European Patent Specification EP 3 793 586 B1, published April 10, 2024. Title: SOLUBLE COMPLEMENT RECEPTOR TYPE 1 VARIANTS AND USES THEREOF. Applicant: CSL Limited CSL Behring AG. The sequence listing filed with the application follows.

SEQUENCE LISTING (51 sequences)

SEQ ID NO: 1 - protein, 1971 aa, Artificial Sequence
  sCR1
MGASSPRSPEPVGPPAPGLPFCCGGSLLAVVVLLALPVAWGQCNAPEWLPFARPTNLTDEFEFPIGTYLNYECRPGYSGRPFSIICLKNSVWTGAKDRCRRKSCRNPPDPVNGMVHVIKGIQFGSQIKYSCTKGYRLIGSSSATCIISGDTVIWDNETPICDRIPCGLPPTITNGDFISTNRENFHYGSVVTYRCNPGSGGRKVFELVGEPSIYCTSNDDQVGIWSGPAPQCIIPNKCTPPNVENGILVSDNRSLFSLNEVVEFRCQPGFVMKGPRRVKCQALNKWEPELPSCSRVCQPPPDVLHAERTQRDKDNFSPGQEVFYSCEPGYDLRGAASMRCTPQGDWSPAAPTCEVKSCDDFMGQLLNGRVLFPVNLQLGAKVDFVCDEGFQLKGSSASYCVLAGMESLWNSSVPVCEQIFCPSPPVIPNGRHTGKPLEVFPFGKTVNYTCDPHPDRGTSFDLIGESTIRCTSDPQGNGVWSSPAPRCGILGHCQAPDHFLFAKLKTQTNASDFPIGTSLKYECRPEYYGRPFSITCLDNLVWSSPKDVCKRKSCKTPPDPVNGMVHVITDIQVGSRINYSCTTGHRLIGHSSAECILSGNAAHWSTKPPICQRIPCGLPPTIANGDFISTNRENFHYGSVVTYRCNPGSGGRKVFELVGEPSIYCTSNDDQVGIWSGPAPQCIIPNKCTPPNVENGILVSDNRSLFSLNEVVEFRCQPGFVMKGPRRVKCQALNKWEPELPSCSRVCQPPPDVLHAERTQRDKDNFSPGQEVFYSCEPGYDLRGAASMRCTPQGDWSPAAPTCEVKSCDDFMGQLLNGRVLFPVNLQLGAKVDFVCDEGFQLKGSSASYCVLAGMESLWNSSVPVCEQIFCPSPPVIPNGRHTGKPLEVFPFGKAVNYTCDPHPDRGTSFDLIGESTIRCTSDPQGNGVWSSPAPRCGILGHCQAPDHFLFAKLKTQTNASDFPIGTSLKYECRPEYYGRPFSITCLDNLVWSSPKDVCKRKSCKTPPDPVNGMVHVITDIQVGSRINYSCTTGHRLIGHSSAECILSGNTAHWSTKPPICQRIPCGLPPTIANGDFISTNRENFHYGSVVTYRCNLGSRGRKVFELVGEPSIYCTSNDDQVGIWSGPAPQCIIPNKCTPPNVENGILVSDNRSLFSLNEVVEFRCQPGFVMKGPRRVKCQALNKWEPELPSCSRVCQPPPEILHGEHTPSHQDNFSPGQEVFYSCEPGYDLRGAASLHCTPQGDWSPEAPRCAVKSCDDFLGQLPHGRVLFPLNLQLGAKVSFVCDEGFRLKGSSVSHCVLVGMRSLWNNSVPVCEHIFCPNPPAILNGRHTGTPSGDIPYGKEISYTCDPHPDRGMTFNLIGESTIRCTSDPHGNGVWSSPAPRCELSVRAGHCKTPEQFPFASPTIPINDFEFPVGTSLNYECRPGYFGKMFSISCLENLVWSSVEDNCRRKSCGPPPEPFNGMVHINTDTQFGSTVNYSCNEGFRLIGSPSTTCLVSGNNVTWDKKAPICEIISCEPPPTISNGDFYSNNRTSFHNGTVVTYQCHTGPDGEQLFELVGERSIYCTSKDDQVGVWSSPPPRCISTNKCTAPEVENAIRVPGNRSFFSLTEIIRFRCQPGFVMVGSHTVQCQTNGRWGPKLPHCSRVCQPPPEILHGEHTLSHQDNFSPGQEVFYSCEPSYDLRGAASLHCTPQGDWSPEAPRCTVKSCDDFLGQLPHGRVLLPLNLQLGAKVSFVCDEGFRLKGRSASHCVLAGMKALWNSSVPVCEQIFCPNPPAILNGRHTGTPFGDIPYGKEISYACDTHPDRGMTFNLIGESSIRCTSDPQGNGVWSSPAPRCELSVPAACPHPPKIQNGHYIGGHVSLYLPGMTISYICDPGYLLVGKGFIFCTDQGIWSQLDHYCKEVNCSFPLFMNGISKELEMKKVYHYGDYVTLKCEDGYTLEGSPWSQCQADDRWDPPLAKCTSRTHD

SEQ ID NO: 2 - protein, 1930 aa, Artificial Sequence
  sCR1(1971)
QCNAPEWLPFARPTNLTDEFEFPIGTYLNYECRPGYSGRPFSIICLKNSVWTGAKDRCRRKSCRNPPDPVNGMVHVIKGIQFGSQIKYSCTKGYRLIGSSSATCIISGDTVIWDNETPICDRIPCGLPPTITNGDFISTNRENFHYGSVVTYRCNPGSGGRKVFELVGEPSIYCTSNDDQVGIWSGPAPQCIIPNKCTPPNVENGILVSDNRSLFSLNEVVEFRCQPGFVMKGPRRVKCQALNKWEPELPSCSRVCQPPPDVLHAERTQRDKDNFSPGQEVFYSCEPGYDLRGAASMRCTPQGDWSPAAPTCEVKSCDDFMGQLLNGRVLFPVNLQLGAKVDFVCDEGFQLKGSSASYCVLAGMESLWNSSVPVCEQIFCPSPPVIPNGRHTGKPLEVFPFGKTVNYTCDPHPDRGTSFDLIGESTIRCTSDPQGNGVWSSPAPRCGILGHCQAPDHFLFAKLKTQTNASDFPIGTSLKYECRPEYYGRPFSITCLDNLVWSSPKDVCKRKSCKTPPDPVNGMVHVITDIQVGSRINYSCTTGHRLIGHSSAECILSGNAAHWSTKPPICQRIPCGLPPTIANGDFISTNRENFHYGSVVTYRCNPGSGGRKVFELVGEPSIYCTSNDDQVGIWSGPAPQCIIPNKCTPPNVENGILVSDNRSLFSLNEVVEFRCQPGFVMKGPRRVKCQALNKWEPELPSCSRVCQPPPDVLHAERTQRDKDNFSPGQEVFYSCEPGYDLRGAASMRCTPQGDWSPAAPTCEVKSCDDFMGQLLNGRVLFPVNLQLGAKVDFVCDEGFQLKGSSASYCVLAGMESLWNSSVPVCEQIFCPSPPVIPNGRHTGKPLEVFPFGKAVNYTCDPHPDRGTSFDLIGESTIRCTSDPQGNGVWSSPAPRCGILGHCQAPDHFLFAKLKTQTNASDFPIGTSLKYECRPEYYGRPFSITCLDNLVWSSPKDVCKRKSCKTPPDPVNGMVHVITDIQVGSRINYSCTTGHRLIGHSSAECILSGNTAHWSTKPPICQRIPCGLPPTIANGDFISTNRENFHYGSVVTYRCNLGSRGRKVFELVGEPSIYCTSNDDQVGIWSGPAPQCIIPNKCTPPNVENGILVSDNRSLFSLNEVVEFRCQPGFVMKGPRRVKCQALNKWEPELPSCSRVCQPPPEILHGEHTPSHQDNFSPGQEVFYSCEPGYDLRGAASLHCTPQGDWSPEAPRCAVKSCDDFLGQLPHGRVLFPLNLQLGAKVSFVCDEGFRLKGSSVSHCVLVGMRSLWNNSVPVCEHIFCPNPPAILNGRHTGTPSGDIPYGKEISYTCDPHPDRGMTFNLIGESTIRCTSDPHGNGVWSSPAPRCELSVRAGHCKTPEQFPFASPTIPINDFEFPVGTSLNYECRPGYFGKMFSISCLENLVWSSVEDNCRRKSCGPPPEPFNGMVHINTDTQFGSTVNYSCNEGFRLIGSPSTTCLVSGNNVTWDKKAPICEIISCEPPPTISNGDFYSNNRTSFHNGTVVTYQCHTGPDGEQLFELVGERSIYCTSKDDQVGVWSSPPPRCISTNKCTAPEVENAIRVPGNRSFFSLTEIIRFRCQPGFVMVGSHTVQCQTNGRWGPKLPHCSRVCQPPPEILHGEHTLSHQDNFSPGQEVFYSCEPSYDLRGAASLHCTPQGDWSPEAPRCTVKSCDDFLGQLPHGRVLLPLNLQLGAKVSFVCDEGFRLKGRSASHCVLAGMKALWNSSVPVCEQIFCPNPPAILNGRHTGTPFGDIPYGKEISYACDTHPDRGMTFNLIGESSIRCTSDPQGNGVWSSPAPRCELSVPAACPHPPKIQNGHYIGGHVSLYLPGMTISYICDPGYLLVGKGFIFCTDQGIWSQLDHYCKEVNCSFPLFMNGISKELEMKKVYHYGDYVTLKCEDGYTLEGSPWSQCQADDRWDPPLAKCTSRTHD

SEQ ID NO: 3 - protein, 1351 aa, Artificial Sequence
  sCR1(1392)
QCNAPEWLPFARPTNLTDEFEFPIGTYLNYECRPGYSGRPFSIICLKNSVWTGAKDRCRRKSCRNPPDPVNGMVHVIKGIQFGSQIKYSCTKGYRLIGSSSATCIISGDTVIWDNETPICDRIPCGLPPTITNGDFISTNRENFHYGSVVTYRCNPGSGGRKVFELVGEPSIYCTSNDDQVGIWSGPAPQCIIPNKCTPPNVENGILVSDNRSLFSLNEVVEFRCQPGFVMKGPRRVKCQALNKWEPELPSCSRVCQPPPDVLHAERTQRDKDNFSPGQEVFYSCEPGYDLRGAASMRCTPQGDWSPAAPTCEVKSCDDFMGQLLNGRVLFPVNLQLGAKVDFVCDEGFQLKGSSASYCVLAGMESLWNSSVPVCEQIFCPSPPVIPNGRHTGKPLEVFPFGKTVNYTCDPHPDRGTSFDLIGESTIRCTSDPQGNGVWSSPAPRCGILGHCQAPDHFLFAKLKTQTNASDFPIGTSLKYECRPEYYGRPFSITCLDNLVWSSPKDVCKRKSCKTPPDPVNGMVHVITDIQVGSRINYSCTTGHRLIGHSSAECILSGNAAHWSTKPPICQRIPCGLPPTIANGDFISTNRENFHYGSVVTYRCNPGSGGRKVFELVGEPSIYCTSNDDQVGIWSGPAPQCIIPNKCTPPNVENGILVSDNRSLFSLNEVVEFRCQPGFVMKGPRRVKCQALNKWEPELPSCSRVCQPPPDVLHAERTQRDKDNFSPGQEVFYSCEPGYDLRGAASMRCTPQGDWSPAAPTCEVKSCDDFMGQLLNGRVLFPVNLQLGAKVDFVCDEGFQLKGSSASYCVLAGMESLWNSSVPVCEQIFCPSPPVIPNGRHTGKPLEVFPFGKAVNYTCDPHPDRGTSFDLIGESTIRCTSDPQGNGVWSSPAPRCGILGHCQAPDHFLFAKLKTQTNASDFPIGTSLKYECRPEYYGRPFSITCLDNLVWSSPKDVCKRKSCKTPPDPVNGMVHVITDIQVGSRINYSCTTGHRLIGHSSAECILSGNTAHWSTKPPICQRIPCGLPPTIANGDFISTNRENFHYGSVVTYRCNLGSRGRKVFELVGEPSIYCTSNDDQVGIWSGPAPQCIIPNKCTPPNVENGILVSDNRSLFSLNEVVEFRCQPGFVMKGPRRVKCQALNKWEPELPSCSRVCQPPPEILHGEHTPSHQDNFSPGQEVFYSCEPGYDLRGAASLHCTPQGDWSPEAPRCAVKSCDDFLGQLPHGRVLFPLNLQLGAKVSFVCDEGFRLKGSSVSHCVLVGMRSLWNNSVPVCEHIFCPNPPAILNGRHTGTPSGDIPYGKEISYTCDPHPDRGMTFNLIGESTIRCTSDPHGNGVWSSPAPRCELSVR

SEQ ID NO: 4 - protein, 898 aa, Artificial Sequence
  sCR1(939)
QCNAPEWLPFARPTNLTDEFEFPIGTYLNYECRPGYSGRPFSIICLKNSVWTGAKDRCRRKSCRNPPDPVNGMVHVIKGIQFGSQIKYSCTKGYRLIGSSSATCIISGDTVIWDNETPICDRIPCGLPPTITNGDFISTNRENFHYGSVVTYRCNPGSGGRKVFELVGEPSIYCTSNDDQVGIWSGPAPQCIIPNKCTPPNVENGILVSDNRSLFSLNEVVEFRCQPGFVMKGPRRVKCQALNKWEPELPSCSRVCQPPPDVLHAERTQRDKDNFSPGQEVFYSCEPGYDLRGAASMRCTPQGDWSPAAPTCEVKSCDDFMGQLLNGRVLFPVNLQLGAKVDFVCDEGFQLKGSSASYCVLAGMESLWNSSVPVCEQIFCPSPPVIPNGRHTGKPLEVFPFGKTVNYTCDPHPDRGTSFDLIGESTIRCTSDPQGNGVWSSPAPRCGILGHCQAPDHFLFAKLKTQTNASDFPIGTSLKYECRPEYYGRPFSITCLDNLVWSSPKDVCKRKSCKTPPDPVNGMVHVITDIQVGSRINYSCTTGHRLIGHSSAECILSGNAAHWSTKPPICQRIPCGLPPTIANGDFISTNRENFHYGSVVTYRCNPGSGGRKVFELVGEPSIYCTSNDDQVGIWSGPAPQCIIPNKCTPPNVENGILVSDNRSLFSLNEVVEFRCQPGFVMKGPRRVKCQALNKWEPELPSCSRVCQPPPDVLHAERTQRDKDNFSPGQEVFYSCEPGYDLRGAASMRCTPQGDWSPAAPTCEVKSCDDFMGQLLNGRVLFPVNLQLGAKVDFVCDEGFQLKGSSASYCVLAGMESLWNSSVPVCEQIFCPSPPVIPNGRHTGKPLEVFPFGKAVNYTCDPHPDRGTSFDLIGESTIRCTSDPQGNGVWSSPAPRCGI

SEQ ID NO: 5 - protein, 903 aa, Artificial Sequence
  sCR1(490-1392)
LGHCQAPDHFLFAKLKTQTNASDFPIGTSLKYECRPEYYGRPFSITCLDNLVWSSPKDVCKRKSCKTPPDPVNGMVHVITDIQVGSRINYSCTTGHRLIGHSSAECILSGNAAHWSTKPPICQRIPCGLPPTIANGDFISTNRENFHYGSVVTYRCNPGSGGRKVFELVGEPSIYCTSNDDQVGIWSGPAPQCIIPNKCTPPNVENGILVSDNRSLFSLNEVVEFRCQPGFVMKGPRRVKCQALNKWEPELPSCSRVCQPPPDVLHAERTQRDKDNFSPGQEVFYSCEPGYDLRGAASMRCTPQGDWSPAAPTCEVKSCDDFMGQLLNGRVLFPVNLQLGAKVDFVCDEGFQLKGSSASYCVLAGMESLWNSSVPVCEQIFCPSPPVIPNGRHTGKPLEVFPFGKAVNYTCDPHPDRGTSFDLIGESTIRCTSDPQGNGVWSSPAPRCGILGHCQAPDHFLFAKLKTQTNASDFPIGTSLKYECRPEYYGRPFSITCLDNLVWSSPKDVCKRKSCKTPPDPVNGMVHVITDIQVGSRINYSCTTGHRLIGHSSAECILSGNTAHWSTKPPICQRIPCGLPPTIANGDFISTNRENFHYGSVVTYRCNLGSRGRKVFELVGEPSIYCTSNDDQVGIWSGPAPQCIIPNKCTPPNVENGILVSDNRSLFSLNEVVEFRCQPGFVMKGPRRVKCQALNKWEPELPSCSRVCQPPPEILHGEHTPSHQDNFSPGQEVFYSCEPGYDLRGAASLHCTPQGDWSPEAPRCAVKSCDDFLGQLPHGRVLFPLNLQLGAKVSFVCDEGFRLKGSSVSHCVLVGMRSLWNNSVPVCEHIFCPNPPAILNGRHTGTPSGDIPYGKEISYTCDPHPDRGMTFNLIGESTIRCTSDPHGNGVWSSPAPRCELSVR

SEQ ID NO: 6 - protein, 1482 aa, Artificial Sequence
  sCR1(490-1971)
LGHCQAPDHFLFAKLKTQTNASDFPIGTSLKYECRPEYYGRPFSITCLDNLVWSSPKDVCKRKSCKTPPDPVNGMVHVITDIQVGSRINYSCTTGHRLIGHSSAECILSGNAAHWSTKPPICQRIPCGLPPTIANGDFISTNRENFHYGSVVTYRCNPGSGGRKVFELVGEPSIYCTSNDDQVGIWSGPAPQCIIPNKCTPPNVENGILVSDNRSLFSLNEVVEFRCQPGFVMKGPRRVKCQALNKWEPELPSCSRVCQPPPDVLHAERTQRDKDNFSPGQEVFYSCEPGYDLRGAASMRCTPQGDWSPAAPTCEVKSCDDFMGQLLNGRVLFPVNLQLGAKVDFVCDEGFQLKGSSASYCVLAGMESLWNSSVPVCEQIFCPSPPVIPNGRHTGKPLEVFPFGKAVNYTCDPHPDRGTSFDLIGESTIRCTSDPQGNGVWSSPAPRCGILGHCQAPDHFLFAKLKTQTNASDFPIGTSLKYECRPEYYGRPFSITCLDNLVWSSPKDVCKRKSCKTPPDPVNGMVHVITDIQVGSRINYSCTTGHRLIGHSSAECILSGNTAHWSTKPPICQRIPCGLPPTIANGDFISTNRENFHYGSVVTYRCNLGSRGRKVFELVGEPSIYCTSNDDQVGIWSGPAPQCIIPNKCTPPNVENGILVSDNRSLFSLNEVVEFRCQPGFVMKGPRRVKCQALNKWEPELPSCSRVCQPPPEILHGEHTPSHQDNFSPGQEVFYSCEPGYDLRGAASLHCTPQGDWSPEAPRCAVKSCDDFLGQLPHGRVLFPLNLQLGAKVSFVCDEGFRLKGSSVSHCVLVGMRSLWNNSVPVCEHIFCPNPPAILNGRHTGTPSGDIPYGKEISYTCDPHPDRGMTFNLIGESTIRCTSDPHGNGVWSSPAPRCELSVRAGHCKTPEQFPFASPTIPINDFEFPVGTSLNYECRPGYFGKMFSISCLENLVWSSVEDNCRRKSCGPPPEPFNGMVHINTDTQFGSTVNYSCNEGFRLIGSPSTTCLVSGNNVTWDKKAPICEIISCEPPPTISNGDFYSNNRTSFHNGTVVTYQCHTGPDGEQLFELVGERSIYCTSKDDQVGVWSSPPPRCISTNKCTAPEVENAIRVPGNRSFFSLTEIIRFRCQPGFVMVGSHTVQCQTNGRWGPKLPHCSRVCQPPPEILHGEHTLSHQDNFSPGQEVFYSCEPSYDLRGAASLHCTPQGDWSPEAPRCTVKSCDDFLGQLPHGRVLLPLNLQLGAKVSFVCDEGFRLKGRSASHCVLAGMKALWNSSVPVCEQIFCPNPPAILNGRHTGTPFGDIPYGKEISYACDTHPDRGMTFNLIGESSIRCTSDPQGNGVWSSPAPRCELSVPAACPHPPKIQNGHYIGGHVSLYLPGMTISYICDPGYLLVGKGFIFCTDQGIWSQLDHYCKEVNCSFPLFMNGISKELEMKKVYHYGDYVTLKCEDGYTLEGSPWSQCQADDRWDPPLAKCTSRTHD

SEQ ID NO: 7 - protein, 193 aa, Artificial Sequence
  sCR1(234)
QCNAPEWLPFARPTNLTDEFEFPIGTYLNYECRPGYSGRPFSIICLKNSVWTGAKDRCRRKSCRNPPDPVNGMVHVIKGIQFGSQIKYSCTKGYRLIGSSSATCIISGDTVIWDNETPICDRIPCGLPPTITNGDFISTNRENFHYGSVVTYRCNPGSGGRKVFELVGEPSIYCTSNDDQVGIWSGPAPQCII

SEQ ID NO: 8 - protein, 448 aa, Artificial Sequence
  sCR1(489)
QCNAPEWLPFARPTNLTDEFEFPIGTYLNYECRPGYSGRPFSIICLKNSVWTGAKDRCRRKSCRNPPDPVNGMVHVIKGIQFGSQIKYSCTKGYRLIGSSSATCIISGDTVIWDNETPICDRIPCGLPPTITNGDFISTNRENFHYGSVVTYRCNPGSGGRKVFELVGEPSIYCTSNDDQVGIWSGPAPQCIIPNKCTPPNVENGILVSDNRSLFSLNEVVEFRCQPGFVMKGPRRVKCQALNKWEPELPSCSRVCQPPPDVLHAERTQRDKDNFSPGQEVFYSCEPGYDLRGAASMRCTPQGDWSPAAPTCEVKSCDDFMGQLLNGRVLFPVNLQLGAKVDFVCDEGFQLKGSSASYCVLAGMESLWNSSVPVCEQIFCPSPPVIPNGRHTGKPLEVFPFGKTVNYTCDPHPDRGTSFDLIGESTIRCTSDPQGNGVWSSPAPRCGI

SEQ ID NO: 9 - protein, 1482 aa, Artificial Sequence; identical to SEQ ID NO: 6
  sCR1(940-1971)

SEQ ID NO: 10 - protein, 450 aa, Artificial Sequence
  sCR1(490-939)
LGHCQAPDHFLFAKLKTQTNASDFPIGTSLKYECRPEYYGRPFSITCLDNLVWSSPKDVCKRKSCKTPPDPVNGMVHVITDIQVGSRINYSCTTGHRLIGHSSAECILSGNAAHWSTKPPICQRIPCGLPPTIANGDFISTNRENFHYGSVVTYRCNPGSGGRKVFELVGEPSIYCTSNDDQVGIWSGPAPQCIIPNKCTPPNVENGILVSDNRSLFSLNEVVEFRCQPGFVMKGPRRVKCQALNKWEPELPSCSRVCQPPPDVLHAERTQRDKDNFSPGQEVFYSCEPGYDLRGAASMRCTPQGDWSPAAPTCEVKSCDDFMGQLLNGRVLFPVNLQLGAKVDFVCDEGFQLKGSSASYCVLAGMESLWNSSVPVCEQIFCPSPPVIPNGRHTGKPLEVFPFGKAVNYTCDPHPDRGTSFDLIGESTIRCTSDPQGNGVWSSPAPRCGI

SEQ ID NO: 11 - protein, 903 aa, Artificial Sequence; identical to SEQ ID NO: 5
  sCR1(940-1392)

SEQ ID NO: 12 - protein, 579 aa, Artificial Sequence
  sCR1(1393-1971)
AGHCKTPEQFPFASPTIPINDFEFPVGTSLNYECRPGYFGKMFSISCLENLVWSSVEDNCRRKSCGPPPEPFNGMVHINTDTQFGSTVNYSCNEGFRLIGSPSTTCLVSGNNVTWDKKAPICEIISCEPPPTISNGDFYSNNRTSFHNGTVVTYQCHTGPDGEQLFELVGERSIYCTSKDDQVGVWSSPPPRCISTNKCTAPEVENAIRVPGNRSFFSLTEIIRFRCQPGFVMVGSHTVQCQTNGRWGPKLPHCSRVCQPPPEILHGEHTLSHQDNFSPGQEVFYSCEPSYDLRGAASLHCTPQGDWSPEAPRCTVKSCDDFLGQLPHGRVLLPLNLQLGAKVSFVCDEGFRLKGRSASHCVLAGMKALWNSSVPVCEQIFCPNPPAILNGRHTGTPFGDIPYGKEISYACDTHPDRGMTFNLIGESSIRCTSDPQGNGVWSSPAPRCELSVPAACPHPPKIQNGHYIGGHVSLYLPGMTISYICDPGYLLVGKGFIFCTDQGIWSQLDHYCKEVNCSFPLFMNGISKELEMKKVYHYGDYVTLKCEDGYTLEGSPWSQCQADDRWDPPLAKCTSRTHD

SEQ ID NO: 13 - protein, 448 aa, Artificial Sequence; identical to SEQ ID NO: 8
  sCR1 LHR-A

SEQ ID NO: 14 - protein, 450 aa, Artificial Sequence; identical to SEQ ID NO: 10
  sCR1 LHR-B

SEQ ID NO: 15 - protein, 453 aa, Artificial Sequence
  sCR1 LHR-C
LGHCQAPDHFLFAKLKTQTNASDFPIGTSLKYECRPEYYGRPFSITCLDNLVWSSPKDVCKRKSCKTPPDPVNGMVHVITDIQVGSRINYSCTTGHRLIGHSSAECILSGNTAHWSTKPPICQRIPCGLPPTIANGDFISTNRENFHYGSVVTYRCNLGSRGRKVFELVGEPSIYCTSNDDQVGIWSGPAPQCIIPNKCTPPNVENGILVSDNRSLFSLNEVVEFRCQPGFVMKGPRRVKCQALNKWEPELPSCSRVCQPPPEILHGEHTPSHQDNFSPGQEVFYSCEPGYDLRGAASLHCTPQGDWSPEAPRCAVKSCDDFLGQLPHGRVLFPLNLQLGAKVSFVCDEGFRLKGSSVSHCVLVGMRSLWNNSVPVCEHIFCPNPPAILNGRHTGTPSGDIPYGKEISYTCDPHPDRGMTFNLIGESTIRCTSDPHGNGVWSSPAPRCELSVR

SEQ ID NO: 16 - protein, 579 aa, Artificial Sequence; identical to SEQ ID NO: 12
  sCR1 LHR-D

SEQ ID NO: 17 - protein, 8 aa, Artificial Sequence
  8xHis Tag
HHHHHHHH

SEQ ID NO: 18 - protein, 41 aa, Artificial Sequence
  endogenous signal peptide
MGASSPRSPEPVGPPAPGLPFCCGGSLLAVVVLLALPVAWG

SEQ ID NO: 19 - protein, 19 aa, Artificial Sequence
  exogenous signal peptide
MKILILGIFLFLCSTPAWA

SEQ ID NO: 20 - protein, 1979 aa, Artificial Sequence
  sCR1(1971)-8His
MGASSPRSPEPVGPPAPGLPFCCGGSLLAVVVLLALPVAWGQCNAPEWLPFARPTNLTDEFEFPIGTYLNYECRPGYSGRPFSIICLKNSVWTGAKDRCRRKSCRNPPDPVNGMVHVIKGIQFGSQIKYSCTKGYRLIGSSSATCIISGDTVIWDNETPICDRIPCGLPPTITNGDFISTNRENFHYGSVVTYRCNPGSGGRKVFELVGEPSIYCTSNDDQVGIWSGPAPQCIIPNKCTPPNVENGILVSDNRSLFSLNEVVEFRCQPGFVMKGPRRVKCQALNKWEPELPSCSRVCQPPPDVLHAERTQRDKDNFSPGQEVFYSCEPGYDLRGAASMRCTPQGDWSPAAPTCEVKSCDDFMGQLLNGRVLFPVNLQLGAKVDFVCDEGFQLKGSSASYCVLAGMESLWNSSVPVCEQIFCPSPPVIPNGRHTGKPLEVFPFGKTVNYTCDPHPDRGTSFDLIGESTIRCTSDPQGNGVWSSPAPRCGILGHCQAPDHFLFAKLKTQTNASDFPIGTSLKYECRPEYYGRPFSITCLDNLVWSSPKDVCKRKSCKTPPDPVNGMVHVITDIQVGSRINYSCTTGHRLIGHSSAECILSGNAAHWSTKPPICQRIPCGLPPTIANGDFISTNRENFHYGSVVTYRCNPGSGGRKVFELVGEPSIYCTSNDDQVGIWSGPAPQCIIPNKCTPPNVENGILVSDNRSLFSLNEVVEFRCQPGFVMKGPRRVKCQALNKWEPELPSCSRVCQPPPDVLHAERTQRDKDNFSPGQEVFYSCEPGYDLRGAASMRCTPQGDWSPAAPTCEVKSCDDFMGQLLNGRVLFPVNLQLGAKVDFVCDEGFQLKGSSASYCVLAGMESLWNSSVPVCEQIFCPSPPVIPNGRHTGKPLEVFPFGKAVNYTCDPHPDRGTSFDLIGESTIRCTSDPQGNGVWSSPAPRCGILGHCQAPDHFLFAKLKTQTNASDFPIGTSLKYECRPEYYGRPFSITCLDNLVWSSPKDVCKRKSCKTPPDPVNGMVHVITDIQVGSRINYSCTTGHRLIGHSSAECILSGNTAHWSTKPPICQRIPCGLPPTIANGDFISTNRENFHYGSVVTYRCNLGSRGRKVFELVGEPSIYCTSNDDQVGIWSGPAPQCIIPNKCTPPNVENGILVSDNRSLFSLNEVVEFRCQPGFVMKGPRRVKCQALNKWEPELPSCSRVCQPPPEILHGEHTPSHQDNFSPGQEVFYSCEPGYDLRGAASLHCTPQGDWSPEAPRCAVKSCDDFLGQLPHGRVLFPLNLQLGAKVSFVCDEGFRLKGSSVSHCVLVGMRSLWNNSVPVCEHIFCPNPPAILNGRHTGTPSGDIPYGKEISYTCDPHPDRGMTFNLIGESTIRCTSDPHGNGVWSSPAPRCELSVRAGHCKTPEQFPFASPTIPINDFEFPVGTSLNYECRPGYFGKMFSISCLENLVWSSVEDNCRRKSCGPPPEPFNGMVHINTDTQFGSTVNYSCNEGFRLIGSPSTTCLVSGNNVTWDKKAPICEIISCEPPPTISNGDFYSNNRTSFHNGTVVTYQCHTGPDGEQLFELVGERSIYCTSKDDQVGVWSSPPPRCISTNKCTAPEVENAIRVPGNRSFFSLTEIIRFRCQPGFVMVGSHTVQCQTNGRWGPKLPHCSRVCQPPPEILHGEHTLSHQDNFSPGQEVFYSCEPSYDLRGAASLHCTPQGDWSPEAPRCTVKSCDDFLGQLPHGRVLLPLNLQLGAKVSFVCDEGFRLKGRSASHCVLAGMKALWNSSVPVCEQIFCPNPPAILNGRHTGTPFGDIPYGKEISYACDTHPDRGMTFNLIGESSIRCTSDPQGNGVWSSPAPRCELSVPAACPHPPKIQNGHYIGGHVSLYLPGMTISYICDPGYLLVGKGFIFCTDQGIWSQLDHYCKEVNCSFPLFMNGISKELEMKKVYHYGDYVTLKCEDGYTLEGSPWSQCQADDRWDPPLAKCTSRTHDHHHHHHHH

SEQ ID NO: 21 - protein, 1400 aa, Artificial Sequence
  sCR1(1392)-8His
MGASSPRSPEPVGPPAPGLPFCCGGSLLAVVVLLALPVAWGQCNAPEWLPFARPTNLTDEFEFPIGTYLNYECRPGYSGRPFSIICLKNSVWTGAKDRCRRKSCRNPPDPVNGMVHVIKGIQFGSQIKYSCTKGYRLIGSSSATCIISGDTVIWDNETPICDRIPCGLPPTITNGDFISTNRENFHYGSVVTYRCNPGSGGRKVFELVGEPSIYCTSNDDQVGIWSGPAPQCIIPNKCTPPNVENGILVSDNRSLFSLNEVVEFRCQPGFVMKGPRRVKCQALNKWEPELPSCSRVCQPPPDVLHAERTQRDKDNFSPGQEVFYSCEPGYDLRGAASMRCTPQGDWSPAAPTCEVKSCDDFMGQLLNGRVLFPVNLQLGAKVDFVCDEGFQLKGSSASYCVLAGMESLWNSSVPVCEQIFCPSPPVIPNGRHTGKPLEVFPFGKTVNYTCDPHPDRGTSFDLIGESTIRCTSDPQGNGVWSSPAPRCGILGHCQAPDHFLFAKLKTQTNASDFPIGTSLKYECRPEYYGRPFSITCLDNLVWSSPKDVCKRKSCKTPPDPVNGMVHVITDIQVGSRINYSCTTGHRLIGHSSAECILSGNAAHWSTKPPICQRIPCGLPPTIANGDFISTNRENFHYGSVVTYRCNPGSGGRKVFELVGEPSIYCTSNDDQVGIWSGPAPQCIIPNKCTPPNVENGILVSDNRSLFSLNEVVEFRCQPGFVMKGPRRVKCQALNKWEPELPSCSRVCQPPPDVLHAERTQRDKDNFSPGQEVFYSCEPGYDLRGAASMRCTPQGDWSPAAPTCEVKSCDDFMGQLLNGRVLFPVNLQLGAKVDFVCDEGFQLKGSSASYCVLAGMESLWNSSVPVCEQIFCPSPPVIPNGRHTGKPLEVFPFGKAVNYTCDPHPDRGTSFDLIGESTIRCTSDPQGNGVWSSPAPRCGILGHCQAPDHFLFAKLKTQTNASDFPIGTSLKYECRPEYYGRPFSITCLDNLVWSSPKDVCKRKSCKTPPDPVNGMVHVITDIQVGSRINYSCTTGHRLIGHSSAECILSGNTAHWSTKPPICQRIPCGLPPTIANGDFISTNRENFHYGSVVTYRCNLGSRGRKVFELVGEPSIYCTSNDDQVGIWSGPAPQCIIPNKCTPPNVENGILVSDNRSLFSLNEVVEFRCQPGFVMKGPRRVKCQALNKWEPELPSCSRVCQPPPEILHGEHTPSHQDNFSPGQEVFYSCEPGYDLRGAASLHCTPQGDWSPEAPRCAVKSCDDFLGQLPHGRVLFPLNLQLGAKVSFVCDEGFRLKGSSVSHCVLVGMRSLWNNSVPVCEHIFCPNPPAILNGRHTGTPSGDIPYGKEISYTCDPHPDRGMTFNLIGESTIRCTSDPHGNGVWSSPAPRCELSVRHHHHHHHH

SEQ ID NO: 22 - protein, 947 aa, Artificial Sequence
  sCR1(939)-8His
MGASSPRSPEPVGPPAPGLPFCCGGSLLAVVVLLALPVAWGQCNAPEWLPFARPTNLTDEFEFPIGTYLNYECRPGYSGRPFSIICLKNSVWTGAKDRCRRKSCRNPPDPVNGMVHVIKGIQFGSQIKYSCTKGYRLIGSSSATCIISGDTVIWDNETPICDRIPCGLPPTITNGDFISTNRENFHYGSVVTYRCNPGSGGRKVFELVGEPSIYCTSNDDQVGIWSGPAPQCIIPNKCTPPNVENGILVSDNRSLFSLNEVVEFRCQPGFVMKGPRRVKCQALNKWEPELPSCSRVCQPPPDVLHAERTQRDKDNFSPGQEVFYSCEPGYDLRGAASMRCTPQGDWSPAAPTCEVKSCDDFMGQLLNGRVLFPVNLQLGAKVDFVCDEGFQLKGSSASYCVLAGMESLWNSSVPVCEQIFCPSPPVIPNGRHTGKPLEVFPFGKTVNYTCDPHPDRGTSFDLIGESTIRCTSDPQGNGVWSSPAPRCGILGHCQAPDHFLFAKLKTQTNASDFPIGTSLKYECRPEYYGRPFSITCLDNLVWSSPKDVCKRKSCKTPPDPVNGMVHVITDIQVGSRINYSCTTGHRLIGHSSAECILSGNAAHWSTKPPICQRIPCGLPPTIANGDFISTNRENFHYGSVVTYRCNPGSGGRKVFELVGEPSIYCTSNDDQVGIWSGPAPQCIIPNKCTPPNVENGILVSDNRSLFSLNEVVEFRCQPGFVMKGPRRVKCQALNKWEPELPSCSRVCQPPPDVLHAERTQRDKDNFSPGQEVFYSCEPGYDLRGAASMRCTPQGDWSPAAPTCEVKSCDDFMGQLLNGRVLFPVNLQLGAKVDFVCDEGFQLKGSSASYCVLAGMESLWNSSVPVCEQIFCPSPPVIPNGRHTGKPLEVFPFGKAVNYTCDPHPDRGTSFDLIGESTIRCTSDPQGNGVWSSPAPRCGIHHHHHHHH

SEQ ID NO: 23 - protein, 930 aa, Artificial Sequence
  sCR1(490-1392)-8His
MKILILGIFLFLCSTPAWALGHCQAPDHFLFAKLKTQTNASDFPIGTSLKYECRPEYYGRPFSITCLDNLVWSSPKDVCKRKSCKTPPDPVNGMVHVITDIQVGSRINYSCTTGHRLIGHSSAECILSGNAAHWSTKPPICQRIPCGLPPTIANGDFISTNRENFHYGSVVTYRCNPGSGGRKVFELVGEPSIYCTSNDDQVGIWSGPAPQCIIPNKCTPPNVENGILVSDNRSLFSLNEVVEFRCQPGFVMKGPRRVKCQALNKWEPELPSCSRVCQPPPDVLHAERTQRDKDNFSPGQEVFYSCEPGYDLRGAASMRCTPQGDWSPAAPTCEVKSCDDFMGQLLNGRVLFPVNLQLGAKVDFVCDEGFQLKGSSASYCVLAGMESLWNSSVPVCEQIFCPSPPVIPNGRHTGKPLEVFPFGKAVNYTCDPHPDRGTSFDLIGESTIRCTSDPQGNGVWSSPAPRCGILGHCQAPDHFLFAKLKTQTNASDFPIGTSLKYECRPEYYGRPFSITCLDNLVWSSPKDVCKRKSCKTPPDPVNGMVHVITDIQVGSRINYSCTTGHRLIGHSSAECILSGNTAHWSTKPPICQRIPCGLPPTIANGDFISTNRENFHYGSVVTYRCNLGSRGRKVFELVGEPSIYCTSNDDQVGIWSGPAPQCIIPNKCTPPNVENGILVSDNRSLFSLNEVVEFRCQPGFVMKGPRRVKCQALNKWEPELPSCSRVCQPPPEILHGEHTPSHQDNFSPGQEVFYSCEPGYDLRGAASLHCTPQGDWSPEAPRCAVKSCDDFLGQLPHGRVLFPLNLQLGAKVSFVCDEGFRLKGSSVSHCVLVGMRSLWNNSVPVCEHIFCPNPPAILNGRHTGTPSGDIPYGKEISYTCDPHPDRGMTFNLIGESTIRCTSDPHGNGVWSSPAPRCELSVRHHHHHHHH

SEQ ID NO: 24 - protein, 1509 aa, Artificial Sequence
  sCR1(490-1971)-8His
MKILILGIFLFLCSTPAWALGHCQAPDHFLFAKLKTQTNASDFPIGTSLKYECRPEYYGRPFSITCLDNLVWSSPKDVCKRKSCKTPPDPVNGMVHVITDIQVGSRINYSCTTGHRLIGHSSAECILSGNAAHWSTKPPICQRIPCGLPPTIANGDFISTNRENFHYGSVVTYRCNPGSGGRKVFELVGEPSIYCTSNDDQVGIWSGPAPQCIIPNKCTPPNVENGILVSDNRSLFSLNEVVEFRCQPGFVMKGPRRVKCQALNKWEPELPSCSRVCQPPPDVLHAERTQRDKDNFSPGQEVFYSCEPGYDLRGAASMRCTPQGDWSPAAPTCEVKSCDDFMGQLLNGRVLFPVNLQLGAKVDFVCDEGFQLKGSSASYCVLAGMESLWNSSVPVCEQIFCPSPPVIPNGRHTGKPLEVFPFGKAVNYTCDPHPDRGTSFDLIGESTIRCTSDPQGNGVWSSPAPRCGILGHCQAPDHFLFAKLKTQTNASDFPIGTSLKYECRPEYYGRPFSITCLDNLVWSSPKDVCKRKSCKTPPDPVNGMVHVITDIQVGSRINYSCTTGHRLIGHSSAECILSGNTAHWSTKPPICQRIPCGLPPTIANGDFISTNRENFHYGSVVTYRCNLGSRGRKVFELVGEPSIYCTSNDDQVGIWSGPAPQCIIPNKCTPPNVENGILVSDNRSLFSLNEVVEFRCQPGFVMKGPRRVKCQALNKWEPELPSCSRVCQPPPEILHGEHTPSHQDNFSPGQEVFYSCEPGYDLRGAASLHCTPQGDWSPEAPRCAVKSCDDFLGQLPHGRVLFPLNLQLGAKVSFVCDEGFRLKGSSVSHCVLVGMRSLWNNSVPVCEHIFCPNPPAILNGRHTGTPSGDIPYGKEISYTCDPHPDRGMTFNLIGESTIRCTSDPHGNGVWSSPAPRCELSVRAGHCKTPEQFPFASPTIPINDFEFPVGTSLNYECRPGYFGKMFSISCLENLVWSSVEDNCRRKSCGPPPEPFNGMVHINTDTQFGSTVNYSCNEGFRLIGSPSTTCLVSGNNVTWDKKAPICEIISCEPPPTISNGDFYSNNRTSFHNGTVVTYQCHTGPDGEQLFELVGERSIYCTSKDDQVGVWSSPPPRCISTNKCTAPEVENAIRVPGNRSFFSLTEIIRFRCQPGFVMVGSHTVQCQTNGRWGPKLPHCSRVCQPPPEILHGEHTLSHQDNFSPGQEVFYSCEPSYDLRGAASLHCTPQGDWSPEAPRCTVKSCDDFLGQLPHGRVLLPLNLQLGAKVSFVCDEGFRLKGRSASHCVLAGMKALWNSSVPVCEQIFCPNPPAILNGRHTGTPFGDIPYGKEISYACDTHPDRGMTFNLIGESSIRCTSDPQGNGVWSSPAPRCELSVPAACPHPPKIQNGHYIGGHVSLYLPGMTISYICDPGYLLVGKGFIFCTDQGIWSQLDHYCKEVNCSFPLFMNGISKELEMKKVYHYGDYVTLKCEDGYTLEGSPWSQCQADDRWDPPLAKCTSRTHDHHHHHHHH

SEQ ID NO: 25 - protein, 242 aa, Artificial Sequence
  sCR1(234)-8His
MGASSPRSPEPVGPPAPGLPFCCGGSLLAVVVLLALPVAWGQCNAPEWLPFARPTNLTDEFEFPIGTYLNYECRPGYSGRPFSIICLKNSVWTGAKDRCRRKSCRNPPDPVNGMVHVIKGIQFGSQIKYSCTKGYRLIGSSSATCIISGDTVIWDNETPICDRIPCGLPPTITNGDFISTNRENFHYGSVVTYRCNPGSGGRKVFELVGEPSIYCTSNDDQVGIWSGPAPQCIIHHHHHHHH

SEQ ID NO: 26 - protein, 497 aa, Artificial Sequence
  sCR1(489)-8His
MGASSPRSPEPVGPPAPGLPFCCGGSLLAVVVLLALPVAWGQCNAPEWLPFARPTNLTDEFEFPIGTYLNYECRPGYSGRPFSIICLKNSVWTGAKDRCRRKSCRNPPDPVNGMVHVIKGIQFGSQIKYSCTKGYRLIGSSSATCIISGDTVIWDNETPICDRIPCGLPPTITNGDFISTNRENFHYGSVVTYRCNPGSGGRKVFELVGEPSIYCTSNDDQVGIWSGPAPQCIIPNKCTPPNVENGILVSDNRSLFSLNEVVEFRCQPGFVMKGPRRVKCQALNKWEPELPSCSRVCQPPPDVLHAERTQRDKDNFSPGQEVFYSCEPGYDLRGAASMRCTPQGDWSPAAPTCEVKSCDDFMGQLLNGRVLFPVNLQLGAKVDFVCDEGFQLKGSSASYCVLAGMESLWNSSVPVCEQIFCPSPPVIPNGRHTGKPLEVFPFGKTVNYTCDPHPDRGTSFDLIGESTIRCTSDPQGNGVWSSPAPRCGIHHHHHHHH

SEQ ID NO: 27 - protein, 1059 aa, Artificial Sequence
  sCR1(940-1971)-8His
MKILILGIFLFLCSTPAWALGHCQAPDHFLFAKLKTQTNASDFPIGTSLKYECRPEYYGRPFSITCLDNLVWSSPKDVCKRKSCKTPPDPVNGMVHVITDIQVGSRINYSCTTGHRLIGHSSAECILSGNTAHWSTKPPICQRIPCGLPPTIANGDFISTNRENFHYGSVVTYRCNLGSRGRKVFELVGEPSIYCTSNDDQVGIWSGPAPQCIIPNKCTPPNVENGILVSDNRSLFSLNEVVEFRCQPGFVMKGPRRVKCQALNKWEPELPSCSRVCQPPPEILHGEHTPSHQDNFSPGQEVFYSCEPGYDLRGAASLHCTPQGDWSPEAPRCAVKSCDDFLGQLPHGRVLFPLNLQLGAKVSFVCDEGFRLKGSSVSHCVLVGMRSLWNNSVPVCEHIFCPNPPAILNGRHTGTPSGDIPYGKEISYTCDPHPDRGMTFNLIGESTIRCTSDPHGNGVWSSPAPRCELSVRAGHCKTPEQFPFASPTIPINDFEFPVGTSLNYECRPGYFGKMFSISCLENLVWSSVEDNCRRKSCGPPPEPFNGMVHINTDTQFGSTVNYSCNEGFRLIGSPSTTCLVSGNNVTWDKKAPICEIISCEPPPTISNGDFYSNNRTSFHNGTVVTYQCHTGPDGEQLFELVGERSIYCTSKDDQVGVWSSPPPRCISTNKCTAPEVENAIRVPGNRSFFSLTEIIRFRCQPGFVMVGSHTVQCQTNGRWGPKLPHCSRVCQPPPEILHGEHTLSHQDNFSPGQEVFYSCEPSYDLRGAASLHCTPQGDWSPEAPRCTVKSCDDFLGQLPHGRVLLPLNLQLGAKVSFVCDEGFRLKGRSASHCVLAGMKALWNSSVPVCEQIFCPNPPAILNGRHTGTPFGDIPYGKEISYACDTHPDRGMTFNLIGESSIRCTSDPQGNGVWSSPAPRCELSVPAACPHPPKIQNGHYIGGHVSLYLPGMTISYICDPGYLLVGKGFIFCTDQGIWSQLDHYCKEVNCSFPLFMNGISKELEMKKVYHYGDYVTLKCEDGYTLEGSPWSQCQADDRWDPPLAKCTSRTHDHHHHHHHH

SEQ ID NO: 28 - protein, 477 aa, Artificial Sequence
  sCR1(490-939)-8His
MKILILGIFLFLCSTPAWALGHCQAPDHFLFAKLKTQTNASDFPIGTSLKYECRPEYYGRPFSITCLDNLVWSSPKDVCKRKSCKTPPDPVNGMVHVITDIQVGSRINYSCTTGHRLIGHSSAECILSGNAAHWSTKPPICQRIPCGLPPTIANGDFISTNRENFHYGSVVTYRCNPGSGGRKVFELVGEPSIYCTSNDDQVGIWSGPAPQCIIPNKCTPPNVENGILVSDNRSLFSLNEVVEFRCQPGFVMKGPRRVKCQALNKWEPELPSCSRVCQPPPDVLHAERTQRDKDNFSPGQEVFYSCEPGYDLRGAASMRCTPQGDWSPAAPTCEVKSCDDFMGQLLNGRVLFPVNLQLGAKVDFVCDEGFQLKGSSASYCVLAGMESLWNSSVPVCEQIFCPSPPVIPNGRHTGKPLEVFPFGKAVNYTCDPHPDRGTSFDLIGESTIRCTSDPQGNGVWSSPAPRCGIHHHHHHHH

SEQ ID NO: 29 - protein, 480 aa, Artificial Sequence
  sCR1(940-1392)-8His
MKILILGIFLFLCSTPAWALGHCQAPDHFLFAKLKTQTNASDFPIGTSLKYECRPEYYGRPFSITCLDNLVWSSPKDVCKRKSCKTPPDPVNGMVHVITDIQVGSRINYSCTTGHRLIGHSSAECILSGNTAHWSTKPPICQRIPCGLPPTIANGDFISTNRENFHYGSVVTYRCNLGSRGRKVFELVGEPSIYCTSNDDQVGIWSGPAPQCIIPNKCTPPNVENGILVSDNRSLFSLNEVVEFRCQPGFVMKGPRRVKCQALNKWEPELPSCSRVCQPPPEILHGEHTPSHQDNFSPGQEVFYSCEPGYDLRGAASLHCTPQGDWSPEAPRCAVKSCDDFLGQLPHGRVLFPLNLQLGAKVSFVCDEGFRLKGSSVSHCVLVGMRSLWNNSVPVCEHIFCPNPPAILNGRHTGTPSGDIPYGKEISYTCDPHPDRGMTFNLIGESTIRCTSDPHGNGVWSSPAPRCELSVRHHHHHHHH

SEQ ID NO: 30 - protein, 606 aa, Artificial Sequence
  sCR1(1393-1971)-8His
MKILILGIFLFLCSTPAWAAGHCKTPEQFPFASPTIPINDFEFPVGTSLNYECRPGYFGKMFSISCLENLVWSSVEDNCRRKSCGPPPEPFNGMVHINTDTQFGSTVNYSCNEGFRLIGSPSTTCLVSGNNVTWDKKAPICEIISCEPPPTISNGDFYSNNRTSFHNGTVVTYQCHTGPDGEQLFELVGERSIYCTSKDDQVGVWSSPPPRCISTNKCTAPEVENAIRVPGNRSFFSLTEIIRFRCQPGFVMVGSHTVQCQTNGRWGPKLPHCSRVCQPPPEILHGEHTLSHQDNFSPGQEVFYSCEPSYDLRGAASLHCTPQGDWSPEAPRCTVKSCDDFLGQLPHGRVLLPLNLQLGAKVSFVCDEGFRLKGRSASHCVLAGMKALWNSSVPVCEQIFCPNPPAILNGRHTGTPFGDIPYGKEISYACDTHPDRGMTFNLIGESSIRCTSDPQGNGVWSSPAPRCELSVPAACPHPPKIQNGHYIGGHVSLYLPGMTISYICDPGYLLVGKGFIFCTDQGIWSQLDHYCKEVNCSFPLFMNGISKELEMKKVYHYGDYVTLKCEDGYTLEGSPWSQCQADDRWDPPLAKCTSRTHDHHHHHHHH

SEQ ID NO: 31 - protein, 13 aa, Artificial Sequence
  Linker
GSGGSGGSGGSGS

SEQ ID NO: 32 - protein, 585 aa, Artificial Sequence [sequence omitted]

SEQ ID NO: 33 - protein, 229 aa, Artificial Sequence
  IgG1 Fc
ESKYGPPCPPCPAPEFLGGPSVFLFPPKPKDTLMISRTPEVTCVVVDVSQEDPEVQFNWYVDGVEVHNAKTKPREEQFNSTYRVVSVLTVLHQDWLNGKEYKCKVSNKGLPSSIEKTISKAKGQPREPQVYTLPPSQEEMTKNQVSLTCLVKGFYPSDAIVEWESNGQPENNYKTTPPVLDSDGSFFLYSRLTVDKSRWQEGNVFSCSVMHEALHNHYTQKSLSLSLGK

SEQ ID NO: 34 - protein, 229 aa, Artificial Sequence
  IgG4 Fc
ESKYGPPCPSCPAPEFLGGPSVFLFPPKPKDTLMISRTPEVTCVVVDVSQEDPEVQFNWYVDGVEVHNAKTKPREEQFNSTYRVVSVLTVLHQDWLNGKEYKCKVSNKGLPSSIEKTISKAKGQPREPQVYTLPPSQEEMTKNQVSLTCLVKGFYPSDIAVEWESNGQPENNYKTTPPVLDSDGSFFLYSRLTVDKSRWQEGNVFSCSVMHEALHNHYTQKSLSLSLGK

SEQ ID NO: 35 - protein, 30 aa, Artificial Sequence
  GS30 peptide linker
SGGSGGSGGSGGSGGSGGSGGSGGSGGSGS

SEQ ID NO: 36 - protein, 18 aa, Artificial Sequence
  exogenous signal peptide
MKWVTFISLLFLFSSAYS

SEQ ID NO: 37 - protein, 19 aa, Artificial Sequence
  exogenous signal peptide
MGWSCIILFLVATATGVHS

SEQ ID NO: 38 - protein, 2569 aa, Artificial Sequence
  amino acid sequence of soluble complement receptor 1 conjugated to HSA (sCR1(1971)-GS13-HSA) with N-terminal endogenous signal peptide
MGASSPRSPEPVGPPAPGLPFCCGGSLLAVVVLLALPVAWGQCNAPEWLPFARPTNLTDEFEFPIGTYLNYECRPGYSGRPFSIICLKNSVWTGAKDRCRRKSCRNPPDPVNGMVHVIKGIQFGSQIKYSCTKGYRLIGSSSATCIISGDTVIWDNETPICDRIPCGLPPTITNGDFISTNRENFHYGSVVTYRCNPGSGGRKVFELVGEPSIYCTSNDDQVGIWSGPAPQCIIPNKCTPPNVENGILVSDNRSLFSLNEVVEFRCQPGFVMKGPRRVKCQALNKWEPELPSCSRVCQPPPDVLHAERTQRDKDNFSPGQEVFYSCEPGYDLRGAASMRCTPQGDWSPAAPTCEVKSCDDFMGQLLNGRVLFPVNLQLGAKVDFVCDEGFQLKGSSASYCVLAGMESLWNSSVPVCEQIFCPSPPVIPNGRHTGKPLEVFPFGKTVNYTCDPHPDRGTSFDLIGESTIRCTSDPQGNGVWSSPAPRCGILGHCQAPDHFLFAKLKTQTNASDFPIGTSLKYECRPEYYGRPFSITCLDNLVWSSPKDVCKRKSCKTPPDPVNGMVHVITDIQVGSRINYSCTTGHRLIGHSSAECILSGNAAHWSTKPPICQRIPCGLPPTIANGDFISTNRENFHYGSVVTYRCNPGSGGRKVFELVGEPSIYCTSNDDQVGIWSGPAPQCIIPNKCTPPNVENGILVSDNRSLFSLNEVVEFRCQPGFVMKGPRRVKCQALNKWEPELPSCSRVCQPPPDVLHAERTQRDKDNFSPGQEVFYSCEPGYDLRGAASMRCTPQGDWSPAAPTCEVKSCDDFMGQLLNGRVLFPVNLQLGAKVDFVCDEGFQLKGSSASYCVLAGMESLWNSSVPVCEQIFCPSPPVIPNGRHTGKPLEVFPFGKAVNYTCDPHPDRGTSFDLIGESTIRCTSDPQGNGVWSSPAPRCGILGHCQAPDHFLFAKLKTQTNASDFPIGTSLKYECRPEYYGRPFSITCLDNLVWSSPKDVCKRKSCKTPPDPVNGMVHVITDIQVGSRINYSCTTGHRLIGHSSAECILSGNTAHWSTKPPICQRIPCGLPPTIANGDFISTNRENFHYGSVVTYRCNLGSRGRKVFELVGEPSIYCTSNDDQVGIWSGPAPQCIIPNKCTPPNVENGILVSDNRSLFSLNEVVEFRCQPGFVMKGPRRVKCQALNKWEPELPSCSRVCQPPPEILHGEHTPSHQDNFSPGQEVFYSCEPGYDLRGAASLHCTPQGDWSPEAPRCAVKSCDDFLGQLPHGRVLFPLNLQLGAKVSFVCDEGFRLKGSSVSHCVLVGMRSLWNNSVPVCEHIFCPNPPAILNGRHTGTPSGDIPYGKEISYTCDPHPDRGMTFNLIGESTIRCTSDPHGNGVWSSPAPRCELSVRAGHCKTPEQFPFASPTIPINDFEFPVGTSLNYECRPGYFGKMFSISCLENLVWSSVEDNCRRKSCGPPPEPFNGMVHINTDTQFGSTVNYSCNEGFRLIGSPSTTCLVSGNNVTWDKKAPICEIISCEPPPTISNGDFYSNNRTSFHNGTVVTYQCHTGPDGEQLFELVGERSIYCTSKDDQVGVWSSPPPRCISTNKCTAPEVENAIRVPGNRSFFSLTEIIRFRCQPGFVMVGSHTVQCQTNGRWGPKLPHCSRVCQPPPEILHGEHTLSHQDNFSPGQEVFYSCEPSYDLRGAASLHCTPQGDWSPEAPRCTVKSCDDFLGQLPHGRVLLPLNLQLGAKVSFVCDEGFRLKGRSASHCVLAGMKALWNSSVPVCEQIFCPNPPAILNGRHTGTPFGDIPYGKEISYACDTHPDRGMTFNLIGESSIRCTSDPQGNGVWSSPAPRCELSVPAACPHPPKIQNGHYIGGHVSLYLPGMTISYICDPGYLLVGKGFIFCTDQGIWSQLDHYCKEVNCSFPLFMNGISKELEMKKVYHYGDYVTLKCEDGYTLEGSPWSQCQADDRWDPPLAKCTSRTHDGSGGSGGSGGSGSDAHKSEVAHRFKDLGEENFKALVLIAFAQYLQQCPFEDHVKLVNEVTEFAKTCVADESAENCDKSLHTLFGDKLCTVATLRETYGEMADCCAKQEPERNECFLQHKDDNPNLPRLVRPEVDVMCTAFHDNEETFLKKYLYEIARRHPYFYAPELLFFAKRYKAAFTECCQAADKAACLLPKLDELRDEGKASSAKQRLKCASLQKFGERAFKAWAVARLSQRFPKAEFAEVSKLVTDLTKVHTECCHGDLLECADDRADLAKYICENQDSISSKLKECCEKPLLEKSHCIAEVENDEMPADLPSLAADFVESKDVCKNYAEAKDVFLGMFLYEYARRHPDYSVVLLLRLAKTYETTLEKCCAAADPHECYAKVFDEFKPLVEEPQNLIKQNCELFEQLGEYKFQNALLVRYTKKVPQVSTPTLVEVSRNLGKVGSKCCKHPEAKRMPCAEDYLSVVLNQLCVLHEKTPVSDRVTKCCTESLVNRRPCFSALEVDETYVPKEFNAETFTFHADICTLSEKERQIKKQTALVELVKHKPKATKEQLKAVMDDFAAFVEKCCKADDKETCFAEEGKKLVAASQAALGL

SEQ ID NO: 39 - protein, 2552 aa, Artificial Sequence
  amino acid sequence of soluble complement receptor 1 conjugated to HSA (HSA-GS13-sCR1(42-1971)) with N-terminal HSA signal peptide and pro-peptide
MKWVTFISLLFLFSSAYSRGVFRRDAHKSEVAHRFKDLGEENFKALVLIAFAQYLQQCPFEDHVKLVNEVTEFAKTCVADESAENCDKSLHTLFGDKLCTVATLRETYGEMADCCAKQEPERNECFLQHKDDNPNLPRLVRPEVDVMCTAFHDNEETFLKKYLYEIARRHPYFYAPELLFFAKRYKAAFTECCQAADKAACLLPKLDELRDEGKASSAKQRLKCASLQKFGERAFKAWAVARLSQRFPKAEFAEVSKLVTDLTKVHTECCHGDLLECADDRADLAKYICENQDSISSKLKECCEKPLLEKSHCIAEVENDEMPADLPSLAADFVESKDVCKNYAEAKDVFLGMFLYEYARRHPDYSVVLLLRLAKTYETTLEKCCAAADPHECYAKVFDEFKPLVEEPQNLIKQNCELFEQLGEYKFQNALLVRYTKKVPQVSTPTLVEVSRNLGKVGSKCCKHPEAKRMPCAEDYLSVVLNQLCVLHEKTPVSDRVTKCCTESLVNRRPCFSALEVDETYVPKEFNAETFTFHADICTLSEKERQIKKQTALVELVKHKPKATKEQLKAVMDDFAAFVEKCCKADDKETCFAEEGKKLVAASQAALGLGSGGSGGSGGSGSQCNAPEWLPFARPTNLTDEFEFPIGTYLNYECRPGYSGRPFSIICLKNSVWTGAKDRCRRKSCRNPPDPVNGMVHVIKGIQFGSQIKYSCTKGYRLIGSSSATCIISGDTVIWDNETPICDRIPCGLPPTITNGDFISTNRENFHYGSVVTYRCNPGSGGRKVFELVGEPSIYCTSNDDQVGIWSGPAPQCIIPNKCTPPNVENGILVSDNRSLFSLNEVVEFRCQPGFVMKGPRRVKCQALNKWEPELPSCSRVCQPPPDVLHAERTQRDKDNFSPGQEVFYSCEPGYDLRGAASMRCTPQGDWSPAAPTCEVKSCDDFMGQLLNGRVLFPVNLQLGAKVDFVCDEGFQLKGSSASYCVLAGMESLWNSSVPVCEQIFCPSPPVIPNGRHTGKPLEVFPFGKTVNYTCDPHPDRGTSFDLIGESTIRCTSDPQGNGVWSSPAPRCGILGHCQAPDHFLFAKLKTQTNASDFPIGTSLKYECRPEYYGRPFSITCLDNLVWSSPKDVCKRKSCKTPPDPVNGMVHVITDIQVGSRINYSCTTGHRLIGHSSAECILSGNAAHWSTKPPICQRIPCGLPPTIANGDFISTNRENFHYGSVVTYRCNPGSGGRKVFELVGEPSIYCTSNDDQVGIWSGPAPQCIIPNKCTPPNVENGILVSDNRSLFSLNEVVEFRCQPGFVMKGPRRVKCQALNKWEPELPSCSRVCQPPPDVLHAERTQRDKDNFSPGQEVFYSCEPGYDLRGAASMRCTPQGDWSPAAPTCEVKSCDDFMGQLLNGRVLFPVNLQLGAKVDFVCDEGFQLKGSSASYCVLAGMESLWNSSVPVCEQIFCPSPPVIPNGRHTGKPLEVFPFGKAVNYTCDPHPDRGTSFDLIGESTIRCTSDPQGNGVWSSPAPRCGILGHCQAPDHFLFAKLKTQTNASDFPIGTSLKYECRPEYYGRPFSITCLDNLVWSSPKDVCKRKSCKTPPDPVNGMVHVITDIQVGSRINYSCTTGHRLIGHSSAECILSGNTAHWSTKPPICQRIPCGLPPTIANGDFISTNRENFHYGSVVTYRCNLGSRGRKVFELVGEPSIYCTSNDDQVGIWSGPAPQCIIPNKCTPPNVENGILVSDNRSLFSLNEVVEFRCQPGFVMKGPRRVKCQALNKWEPELPSCSRVCQPPPEILHGEHTPSHQDNFSPGQEVFYSCEPGYDLRGAASLHCTPQGDWSPEAPRCAVKSCDDFLGQLPHGRVLFPLNLQLGAKVSFVCDEGFRLKGSSVSHCVLVGMRSLWNNSVPVCEHIFCPNPPAILNGRHTGTPSGDIPYGKEISYTCDPHPDRGMTFNLIGESTIRCTSDPHGNGVWSSPAPRCELSVRAGHCKTPEQFPFASPTIPINDFEFPVGTSLNYECRPGYFGKMFSISCLENLVWSSVEDNCRRKSCGPPPEPFNGMVHINTDTQFGSTVNYSCNEGFRLIGSPSTTCLVSGNNVTWDKKAPICEIISCEPPPTISNGDFYSNNRTSFHNGTVVTYQCHTGPDGEQLFELVGERSIYCTSKDDQVGVWSSPPPRCISTNKCTAPEVENAIRVPGNRSFFSLTEIIRFRCQPGFVMVGSHTVQCQTNGRWGPKLPHCSRVCQPPPEILHGEHTLSHQDNFSPGQEVFYSCEPSYDLRGAASLHCTPQGDWSPEAPRCTVKSCDDFLGQLPHGRVLLPLNLQLGAKVSFVCDEGFRLKGRSASHCVLAGMKALWNSSVPVCEQIFCPNPPAILNGRHTGTPFGDIPYGKEISYACDTHPDRGMTFNLIGESSIRCTSDPQGNGVWSSPAPRCELSVPAACPHPPKIQNGHYIGGHVSLYLPGMTISYICDPGYLLVGKGFIFCTDQGIWSQLDHYCKEVNCSFPLFMNGISKELEMKKVYHYGDYVTLKCEDGYTLEGSPWSQCQADDRWDPPLAKCTSRTHD

SEQ ID NO: 40 - protein, 2200 aa, Artificial Sequence
  sCR1(1971)-IgG4 Fc
MGASSPRSPEPVGPPAPGLPFCCGGSLLAVVVLLALPVAWGQCNAPEWLPFARPTNLTDEFEFPIGTYLNYECRPGYSGRPFSIICLKNSVWTGAKDRCRRKSCRNPPDPVNGMVHVIKGIQFGSQIKYSCTKGYRLIGSSSATCIISGDTVIWDNETPICDRIPCGLPPTITNGDFISTNRENFHYGSVVTYRCNPGSGGRKVFELVGEPSIYCTSNDDQVGIWSGPAPQCIIPNKCTPPNVENGILVSDNRSLFSLNEVVEFRCQPGFVMKGPRRVKCQALNKWEPELPSCSRVCQPPPDVLHAERTQRDKDNFSPGQEVFYSCEPGYDLRGAASMRCTPQGDWSPAAPTCEVKSCDDFMGQLLNGRVLFPVNLQLGAKVDFVCDEGFQLKGSSASYCVLAGMESLWNSSVPVCEQIFCPSPPVIPNGRHTGKPLEVFPFGKTVNYTCDPHPDRGTSFDLIGESTIRCTSDPQGNGVWSSPAPRCGILGHCQAPDHFLFAKLKTQTNASDFPIGTSLKYECRPEYYGRPFSITCLDNLVWSSPKDVCKRKSCKTPPDPVNGMVHVITDIQVGSRINYSCTTGHRLIGHSSAECILSGNAAHWSTKPPICQRIPCGLPPTIANGDFISTNRENFHYGSVVTYRCNPGSGGRKVFELVGEPSIYCTSNDDQVGIWSGPAPQCIIPNKCTPPNVENGILVSDNRSLFSLNEVVEFRCQPGFVMKGPRRVKCQALNKWEPELPSCSRVCQPPPDVLHAERTQRDKDNFSPGQEVFYSCEPGYDLRGAASMRCTPQGDWSPAAPTCEVKSCDDFMGQLLNGRVLFPVNLQLGAKVDFVCDEGFQLKGSSASYCVLAGMESLWNSSVPVCEQIFCPSPPVIPNGRHTGKPLEVFPFGKAVNYTCDPHPDRGTSFDLIGESTIRCTSDPQGNGVWSSPAPRCGILGHCQAPDHFLFAKLKTQTNASDFPIGTSLKYECRPEYYGRPFSITCLDNLVWSSPKDVCKRKSCKTPPDPVNGMVHVITDIQVGSRINYSCTTGHRLIGHSSAECILSGNTAHWSTKPPICQRIPCGLPPTIANGDFISTNRENFHYGSVVTYRCNLGSRGRKVFELVGEPSIYCTSNDDQVGIWSGPAPQCIIPNKCTPPNVENGILVSDNRSLFSLNEVVEFRCQPGFVMKGPRRVKCQALNKWEPELPSCSRVCQPPPEILHGEHTPSHQDNFSPGQEVFYSCEPGYDLRGAASLHCTPQGDWSPEAPRCAVKSCDDFLGQLPHGRVLFPLNLQLGAKVSFVCDEGFRLKGSSVSHCVLVGMRSLWNNSVPVCEHIFCPNPPAILNGRHTGTPSGDIPYGKEISYTCDPHPDRGMTFNLIGESTIRCTSDPHGNGVWSSPAPRCELSVRAGHCKTPEQFPFASPTIPINDFEFPVGTSLNYECRPGYFGKMFSISCLENLVWSSVEDNCRRKSCGPPPEPFNGMVHINTDTQFGSTVNYSCNEGFRLIGSPSTTCLVSGNNVTWDKKAPICEIISCEPPPTISNGDFYSNNRTSFHNGTVVTYQCHTGPDGEQLFELVGERSIYCTSKDDQVGVWSSPPPRCISTNKCTAPEVENAIRVPGNRSFFSLTEIIRFRCQPGFVMVGSHTVQCQTNGRWGPKLPHCSRVCQPPPEILHGEHTLSHQDNFSPGQEVFYSCEPSYDLRGAASLHCTPQGDWSPEAPRCTVKSCDDFLGQLPHGRVLLPLNLQLGAKVSFVCDEGFRLKGRSASHCVLAGMKALWNSSVPVCEQIFCPNPPAILNGRHTGTPFGDIPYGKEISYACDTHPDRGMTFNLIGESSIRCTSDPQGNGVWSSPAPRCELSVPAACPHPPKIQNGHYIGGHVSLYLPGMTISYICDPGYLLVGKGFIFCTDQGIWSQLDHYCKEVNCSFPLFMNGISKELEMKKVYHYGDYVTLKCEDGYTLEGSPWSQCQADDRWDPPLAKCTSRTHDESKYGPPCPPCPAPEFLGGPSVFLFPPKPKDTLMISRTPEVTCVVVDVSQEDPEVQFNWYVDGVEVHNAKTKPREEQFNSTYRVVSVLTVLHQDWLNGKEYKCKVSNKGLPSSIEKTISKAKGQPREPQVYTLPPSQEEMTKNQVSLTCLVKGFYPSDAIVEWESNGQPENNYKTTPPVLDSDGSFFLYSRLTVDKSRWQEGNVFSCSVMHEALHNHYTQKSLSLSLGK

SEQ ID NO: 41 - protein, 2178 aa, Artificial Sequence
  IgG4 Fc-sCR1(1971)
MGWSCIILFLVATATGVHSESKYGPPCPSCPAPEFLGGPSVFLFPPKPKDTLMISRTPEVTCVVVDVSQEDPEVQFNWYVDGVEVHNAKTKPREEQFNSTYRVVSVLTVLHQDWLNGKEYKCKVSNKGLPSSIEKTISKAKGQPREPQVYTLPPSQEEMTKNQVSLTCLVKGFYPSDIAVEWESNGQPENNYKTTPPVLDSDGSFFLYSRLTVDKSRWQEGNVFSCSVMHEALHNHYTQKSLSLSLGKQCNAPEWLPFARPTNLTDEFEFPIGTYLNYECRPGYSGRPFSIICLKNSVWTGAKDRCRRKSCRNPPDPVNGMVHVIKGIQFGSQIKYSCTKGYRLIGSSSATCIISGDTVIWDNETPICDRIPCGLPPTITNGDFISTNRENFHYGSVVTYRCNPGSGGRKVFELVGEPSIYCTSNDDQVGIWSGPAPQCIIPNKCTPPNVENGILVSDNRSLFSLNEVVEFRCQPGFVMKGPRRVKCQALNKWEPELPSCSRVCQPPPDVLHAERTQRDKDNFSPGQEVFYSCEPGYDLRGAASMRCTPQGDWSPAAPTCEVKSCDDFMGQLLNGRVLFPVNLQLGAKVDFVCDEGFQLKGSSASYCVLAGMESLWNSSVPVCEQIFCPSPPVIPNGRHTGKPLEVFPFGKTVNYTCDPHPDRGTSFDLIGESTIRCTSDPQGNGVWSSPAPRCGILGHCQAPDHFLFAKLKTQTNASDFPIGTSLKYECRPEYYGRPFSITCLDNLVWSSPKDVCKRKSCKTPPDPVNGMVHVITDIQVGSRINYSCTTGHRLIGHSSAECILSGNAAHWSTKPPICQRIPCGLPPTIANGDFISTNRENFHYGSVVTYRCNPGSGGRKVFELVGEPSIYCTSNDDQVGIWSGPAPQCIIPNKCTPPNVENGILVSDNRSLFSLNEVVEFRCQPGFVMKGPRRVKCQALNKWEPELPSCSRVCQPPPDVLHAERTQRDKDNFSPGQEVFYSCEPGYDLRGAASMRCTPQGDWSPAAPTCEVKSCDDFMGQLLNGRVLFPVNLQLGAKVDFVCDEGFQLKGSSASYCVLAGMESLWNSSVPVCEQIFCPSPPVIPNGRHTGKPLEVFPFGKAVNYTCDPHPDRGTSFDLIGESTIRCTSDPQGNGVWSSPAPRCGILGHCQAPDHFLFAKLKTQTNASDFPIGTSLKYECRPEYYGRPFSITCLDNLVWSSPKDVCKRKSCKTPPDPVNGMVHVITDIQVGSRINYSCTTGHRLIGHSSAECILSGNTAHWSTKPPICQRIPCGLPPTIANGDFISTNRENFHYGSVVTYRCNLGSRGRKVFELVGEPSIYCTSNDDQVGIWSGPAPQCIIPNKCTPPNVENGILVSDNRSLFSLNEVVEFRCQPGFVMKGPRRVKCQALNKWEPELPSCSRVCQPPPEILHGEHTPSHQDNFSPGQEVFYSCEPGYDLRGAASLHCTPQGDWSPEAPRCAVKSCDDFLGQLPHGRVLFPLNLQLGAKVSFVCDEGFRLKGSSVSHCVLVGMRSLWNNSVPVCEHIFCPNPPAILNGRHTGTPSGDIPYGKEISYTCDPHPDRGMTFNLIGESTIRCTSDPHGNGVWSSPAPRCELSVRAGHCKTPEQFPFASPTIPINDFEFPVGTSLNYECRPGYFGKMFSISCLENLVWSSVEDNCRRKSCGPPPEPFNGMVHINTDTQFGSTVNYSCNEGFRLIGSPSTTCLVSGNNVTWDKKAPICEIISCEPPPTISNGDFYSNNRTSFHNGTVVTYQCHTGPDGEQLFELVGERSIYCTSKDDQVGVWSSPPPRCISTNKCTAPEVENAIRVPGNRSFFSLTEIIRFRCQPGFVMVGSHTVQCQTNGRWGPKLPHCSRVCQPPPEILHGEHTLSHQDNFSPGQEVFYSCEPSYDLRGAASLHCTPQGDWSPEAPRCTVKSCDDFLGQLPHGRVLLPLNLQLGAKVSFVCDEGFRLKGRSASHCVLAGMKALWNSSVPVCEQIFCPNPPAILNGRHTGTPFGDIPYGKEISYACDTHPDRGMTFNLIGESSIRCTSDPQGNGVWSSPAPRCELSVPAACPHPPKIQNGHYIGGHVSLYLPGMTISYICDPGYLLVGKGFIFCTDQGIWSQLDHYCKEVNCSFPLFMNGISKELEMKKVYHYGDYVTLKCEDGYTLEGSPWSQCQADDRWDPPLAKCTSRTHD

SEQ ID NO: 42 - protein, 6 aa, Artificial Sequence
  amino acid sequence of HSA pro-peptide
RGVFRR

SEQ ID NO: 43 - protein, 1990 aa, Artificial Sequence
  sCR1(1392)-GS-HSA
MGASSPRSPEPVGPPAPGLPFCCGGSLLAVVVLLALPVAWGQCNAPEWLPFARPTNLTDEFEFPIGTYLNYECRPGYSGRPFSIICLKNSVWTGAKDRCRRKSCRNPPDPVNGMVHVIKGIQFGSQIKYSCTKGYRLIGSSSATCIISGDTVIWDNETPICDRIPCGLPPTITNGDFISTNRENFHYGSVVTYRCNPGSGGRKVFELVGEPSIYCTSNDDQVGIWSGPAPQCIIPNKCTPPNVENGILVSDNRSLFSLNEVVEFRCQPGFVMKGPRRVKCQALNKWEPELPSCSRVCQPPPDVLHAERTQRDKDNFSPGQEVFYSCEPGYDLRGAASMRCTPQGDWSPAAPTCEVKSCDDFMGQLLNGRVLFPVNLQLGAKVDFVCDEGFQLKGSSASYCVLAGMESLWNSSVPVCEQIFCPSPPVIPNGRHTGKPLEVFPFGKTVNYTCDPHPDRGTSFDLIGESTIRCTSDPQGNGVWSSPAPRCGILGHCQAPDHFLFAKLKTQTNASDFPIGTSLKYECRPEYYGRPFSITCLDNLVWSSPKDVCKRKSCKTPPDPVNGMVHVITDIQVGSRINYSCTTGHRLIGHSSAECILSGNAAHWSTKPPICQRIPCGLPPTIANGDFISTNRENFHYGSVVTYRCNPGSGGRKVFELVGEPSIYCTSNDDQVGIWSGPAPQCIIPNKCTPPNVENGILVSDNRSLFSLNEVVEFRCQPGFVMKGPRRVKCQALNKWEPELPSCSRVCQPPPDVLHAERTQRDKDNFSPGQEVFYSCEPGYDLRGAASMRCTPQGDWSPAAPTCEVKSCDDFMGQLLNGRVLFPVNLQLGAKVDFVCDEGFQLKGSSASYCVLAGMESLWNSSVPVCEQIFCPSPPVIPNGRHTGKPLEVFPFGKAVNYTCDPHPDRGTSFDLIGESTIRCTSDPQGNGVWSSPAPRCGILGHCQAPDHFLFAKLKTQTNASDFPIGTSLKYECRPEYYGRPFSITCLDNLVWSSPKDVCKRKSCKTPPDPVNGMVHVITDIQVGSRINYSCTTGHRLIGHSSAECILSGNTAHWSTKPPICQRIPCGLPPTIANGDFISTNRENFHYGSVVTYRCNLGSRGRKVFELVGEPSIYCTSNDDQVGIWSGPAPQCIIPNKCTPPNVENGILVSDNRSLFSLNEVVEFRCQPGFVMKGPRRVKCQALNKWEPELPSCSRVCQPPPEILHGEHTPSHQDNFSPGQEVFYSCEPGYDLRGAASLHCTPQGDWSPEAPRCAVKSCDDFLGQLPHGRVLFPLNLQLGAKVSFVCDEGFRLKGSSVSHCVLVGMRSLWNNSVPVCEHIFCPNPPAILNGRHTGTPSGDIPYGKEISYTCDPHPDRGMTFNLIGESTIRCTSDPHGNGVWSSPAPRCELSVRGSGGSGGSGGSGSDAHKSEVAHRFKDLGEENFKALVLIAFAQYLQQCPFEDHVKLVNEVTEFAKTCVADESAENCDKSLHTLFGDKLCTVATLRETYGEMADCCAKQEPERNECFLQHKDDNPNLPRLVRPEVDVMCTAFHDNEETFLKKYLYEIARRHPYFYAPELLFFAKRYKAAFTECCQAADKAACLLPKLDELRDEGKASSAKQRLKCASLQKFGERAFKAWAVARLSQRFPKAEFAEVSKLVTDLTKVHTECCHGDLLECADDRADLAKYICENQDSISSKLKECCEKPLLEKSHCIAEVENDEMPADLPSLAADFVESKDVCKNYAEAKDVFLGMFLYEYARRHPDYSVVLLLRLAKTYETTLEKCCAAADPHECYAKVFDEFKPLVEEPQNLIKQNCELFEQLGEYKFQNALLVRYTKKVPQVSTPTLVEVSRNLGKVGSKCCKHPEAKRMPCAEDYLSVVLNQLCVLHEKTPVSDRVTKCCTESLVNRRPCFSALEVDETYVPKEFNAETFTFHADICTLSEKERQIKKQTALVELVKHKPKATKEQLKAVMDDFAAFVEKCCKADDKETCFAEEGKKLVAASQAALGL

SEQ ID NO: 44 - protein, 1973 aa, Artificial Sequence
  HSA-GS-sCR1(1392)
MKWVTFISLLFLFSSAYSRGVFRRDAHKSEVAHRFKDLGEENFKALVLIAFAQYLQQCPFEDHVKLVNEVTEFAKTCVADESAENCDKSLHTLFGDKLCTVATLRETYGEMADCCAKQEPERNECFLQHKDDNPNLPRLVRPEVDVMCTAFHDNEETFLKKYLYEIARRHPYFYAPELLFFAKRYKAAFTECCQAADKAACLLPKLDELRDEGKASSAKQRLKCASLQKFGERAFKAWAVARLSQRFPKAEFAEVSKLVTDLTKVHTECCHGDLLECADDRADLAKYICENQDSISSKLKECCEKPLLEKSHCIAEVENDEMPADLPSLAADFVESKDVCKNYAEAKDVFLGMFLYEYARRHPDYSVVLLLRLAKTYETTLEKCCAAADPHECYAKVFDEFKPLVEEPQNLIKQNCELFEQLGEYKFQNALLVRYTKKVPQVSTPTLVEVSRNLGKVGSKCCKHPEAKRMPCAEDYLSVVLNQLCVLHEKTPVSDRVTKCCTESLVNRRPCFSALEVDETYVPKEFNAETFTFHADICTLSEKERQIKKQTALVELVKHKPKATKEQLKAVMDDFAAFVEKCCKADDKETCFAEEGKKLVAASQAALGLGSGGSGGSGGSGSQCNAPEWLPFARPTNLTDEFEFPIGTYLNYECRPGYSGRPFSIICLKNSVWTGAKDRCRRKSCRNPPDPVNGMVHVIKGIQFGSQIKYSCTKGYRLIGSSSATCIISGDTVIWDNETPICDRIPCGLPPTITNGDFISTNRENFHYGSVVTYRCNPGSGGRKVFELVGEPSIYCTSNDDQVGIWSGPAPQCIIPNKCTPPNVENGILVSDNRSLFSLNEVVEFRCQPGFVMKGPRRVKCQALNKWEPELPSCSRVCQPPPDVLHAERTQRDKDNFSPGQEVFYSCEPGYDLRGAASMRCTPQGDWSPAAPTCEVKSCDDFMGQLLNGRVLFPVNLQLGAKVDFVCDEGFQLKGSSASYCVLAGMESLWNSSVPVCEQIFCPSPPVIPNGRHTGKPLEVFPFGKTVNYTCDPHPDRGTSFDLIGESTIRCTSDPQGNGVWSSPAPRCGILGHCQAPDHFLFAKLKTQTNASDFPIGTSLKYECRPEYYGRPFSITCLDNLVWSSPKDVCKRKSCKTPPDPVNGMVHVITDIQVGSRINYSCTTGHRLIGHSSAECILSGNAAHWSTKPPICQRIPCGLPPTIANGDFISTNRENFHYGSVVTYRCNPGSGGRKVFELVGEPSIYCTSNDDQVGIWSGPAPQCIIPNKCTPPNVENGILVSDNRSLFSLNEVVEFRCQPGFVMKGPRRVKCQALNKWEPELPSCSRVCQPPPDVLHAERTQRDKDNFSPGQEVFYSCEPGYDLRGAASMRCTPQGDWSPAAPTCEVKSCDDFMGQLLNGRVLFPVNLQLGAKVDFVCDEGFQLKGSSASYCVLAGMESLWNSSVPVCEQIFCPSPPVIPNGRHTGKPLEVFPFGKAVNYTCDPHPDRGTSFDLIGESTIRCTSDPQGNGVWSSPAPRCGILGHCQAPDHFLFAKLKTQTNASDFPIGTSLKYECRPEYYGRPFSITCLDNLVWSSPKDVCKRKSCKTPPDPVNGMVHVITDIQVGSRINYSCTTGHRLIGHSSAECILSGNTAHWSTKPPICQRIPCGLPPTIANGDFISTNRENFHYGSVVTYRCNLGSRGRKVFELVGEPSIYCTSNDDQVGIWSGPAPQCIIPNKCTPPNVENGILVSDNRSLFSLNEVVEFRCQPGFVMKGPRRVKCQALNKWEPELPSCSRVCQPPPEILHGEHTPSHQDNFSPGQEVFYSCEPGYDLRGAASLHCTPQGDWSPEAPRCAVKSCDDFLGQLPHGRVLFPLNLQLGAKVSFVCDEGFRLKGSSVSHCVLVGMRSLWNNSVPVCEHIFCPNPPAILNGRHTGTPSGDIPYGKEISYTCDPHPDRGMTFNLIGESTIRCTSDPHGNGVWSSPAPRCELSVR

SEQ ID NO: 45 - protein, 1621 aa, Artificial Sequence
  sCR1(1392)-IgG1 Fc
MGASSPRSPEPVGPPAPGLPFCCGGSLLAVVVLLALPVAWGQCNAPEWLPFARPTNLTDEFEFPIGTYLNYECRPGYSGRPFSIICLKNSVWTGAKDRCRRKSCRNPPDPVNGMVHVIKGIQFGSQIKYSCTKGYRLIGSSSATCIISGDTVIWDNETPICDRIPCGLPPTITNGDFISTNRENFHYGSVVTYRCNPGSGGRKVFELVGEPSIYCTSNDDQVGIWSGPAPQCIIPNKCTPPNVENGILVSDNRSLFSLNEVVEFRCQPGFVMKGPRRVKCQALNKWEPELPSCSRVCQPPPDVLHAERTQRDKDNFSPGQEVFYSCEPGYDLRGAASMRCTPQGDWSPAAPTCEVKSCDDFMGQLLNGRVLFPVNLQLGAKVDFVCDEGFQLKGSSASYCVLAGMESLWNSSVPVCEQIFCPSPPVIPNGRHTGKPLEVFPFGKTVNYTCDPHPDRGTSFDLIGESTIRCTSDPQGNGVWSSPAPRCGILGHCQAPDHFLFAKLKTQTNASDFPIGTSLKYECRPEYYGRPFSITCLDNLVWSSPKDVCKRKSCKTPPDPVNGMVHVITDIQVGSRINYSCTTGHRLIGHSSAECILSGNAAHWSTKPPICQRIPCGLPPTIANGDFISTNRENFHYGSVVTYRCNPGSGGRKVFELVGEPSIYCTSNDDQVGIWSGPAPQCIIPNKCTPPNVENGILVSDNRSLFSLNEVVEFRCQPGFVMKGPRRVKCQALNKWEPELPSCSRVCQPPPDVLHAERTQRDKDNFSPGQEVFYSCEPGYDLRGAASMRCTPQGDWSPAAPTCEVKSCDDFMGQLLNGRVLFPVNLQLGAKVDFVCDEGFQLKGSSASYCVLAGMESLWNSSVPVCEQIFCPSPPVIPNGRHTGKPLEVFPFGKAVNYTCDPHPDRGTSFDLIGESTIRCTSDPQGNGVWSSPAPRCGILGHCQAPDHFLFAKLKTQTNASDFPIGTSLKYECRPEYYGRPFSITCLDNLVWSSPKDVCKRKSCKTPPDPVNGMVHVITDIQVGSRINYSCTTGHRLIGHSSAECILSGNTAHWSTKPPICQRIPCGLPPTIANGDFISTNRENFHYGSVVTYRCNLGSRGRKVFELVGEPSIYCTSNDDQVGIWSGPAPQCIIPNKCTPPNVENGILVSDNRSLFSLNEVVEFRCQPGFVMKGPRRVKCQALNKWEPELPSCSRVCQPPPEILHGEHTPSHQDNFSPGQEVFYSCEPGYDLRGAASLHCTPQGDWSPEAPRCAVKSCDDFLGQLPHGRVLFPLNLQLGAKVSFVCDEGFRLKGSSVSHCVLVGMRSLWNNSVPVCEHIFCPNPPAILNGRHTGTPSGDIPYGKEISYTCDPHPDRGMTFNLIGESTIRCTSDPHGNGVWSSPAPRCELSVRESKYGPPCPPCPAPEFLGGPSVFLFPPKPKDTLMISRTPEVTCVVVDVSQEDPEVQFNWYVDGVEVHNAKTKPREEQFNSTYRVVSVLTVLHQDWLNGKEYKCKVSNKGLPSSIEKTISKAKGQPREPQVYTLPPSQEEMTKNQVSLTCLVKGFYPSDAIVEWESNGQPENNYKTTPPVLDSDGSFFLYSRLTVDKSRWQEGNVFSCSVMHEALHNHYTQKSLSLSLGK

SEQ ID NO: 46 - protein, 1621 aa, Artificial Sequence; identical to SEQ ID NO: 45
  amino acid sequence of truncated mature soluble complement receptor 1 conjugated to IgG4 Fc (sCR1(1392)-IgG4 Fc) with N-terminal endogenous signal peptide

SEQ ID NO: 47 - protein, 1599 aa, Artificial Sequence
  IgG4 Fc-sCR1(1392)
MGWSCIILFLVATATGVHSESKYGPPCPSCPAPEFLGGPSVFLFPPKPKDTLMISRTPEVTCVVVDVSQEDPEVQFNWYVDGVEVHNAKTKPREEQFNSTYRVVSVLTVLHQDWLNGKEYKCKVSNKGLPSSIEKTISKAKGQPREPQVYTLPPSQEEMTKNQVSLTCLVKGFYPSDIAVEWESNGQPENNYKTTPPVLDSDGSFFLYSRLTVDKSRWQEGNVFSCSVMHEALHNHYTQKSLSLSLGKQCNAPEWLPFARPTNLTDEFEFPIGTYLNYECRPGYSGRPFSIICLKNSVWTGAKDRCRRKSCRNPPDPVNGMVHVIKGIQFGSQIKYSCTKGYRLIGSSSATCIISGDTVIWDNETPICDRIPCGLPPTITNGDFISTNRENFHYGSVVTYRCNPGSGGRKVFELVGEPSIYCTSNDDQVGIWSGPAPQCIIPNKCTPPNVENGILVSDNRSLFSLNEVVEFRCQPGFVMKGPRRVKCQALNKWEPELPSCSRVCQPPPDVLHAERTQRDKDNFSPGQEVFYSCEPGYDLRGAASMRCTPQGDWSPAAPTCEVKSCDDFMGQLLNGRVLFPVNLQLGAKVDFVCDEGFQLKGSSASYCVLAGMESLWNSSVPVCEQIFCPSPPVIPNGRHTGKPLEVFPFGKTVNYTCDPHPDRGTSFDLIGESTIRCTSDPQGNGVWSSPAPRCGILGHCQAPDHFLFAKLKTQTNASDFPIGTSLKYECRPEYYGRPFSITCLDNLVWSSPKDVCKRKSCKTPPDPVNGMVHVITDIQVGSRINYSCTTGHRLIGHSSAECILSGNAAHWSTKPPICQRIPCGLPPTIANGDFISTNRENFHYGSVVTYRCNPGSGGRKVFELVGEPSIYCTSNDDQVGIWSGPAPQCIIPNKCTPPNVENGILVSDNRSLFSLNEVVEFRCQPGFVMKGPRRVKCQALNKWEPELPSCSRVCQPPPDVLHAERTQRDKDNFSPGQEVFYSCEPGYDLRGAASMRCTPQGDWSPAAPTCEVKSCDDFMGQLLNGRVLFPVNLQLGAKVDFVCDEGFQLKGSSASYCVLAGMESLWNSSVPVCEQIFCPSPPVIPNGRHTGKPLEVFPFGKAVNYTCDPHPDRGTSFDLIGESTIRCTSDPQGNGVWSSPAPRCGILGHCQAPDHFLFAKLKTQTNASDFPIGTSLKYECRPEYYGRPFSITCLDNLVWSSPKDVCKRKSCKTPPDPVNGMVHVITDIQVGSRINYSCTTGHRLIGHSSAECILSGNTAHWSTKPPICQRIPCGLPPTIANGDFISTNRENFHYGSVVTYRCNLGSRGRKVFELVGEPSIYCTSNDDQVGIWSGPAPQCIIPNKCTPPNVENGILVSDNRSLFSLNEVVEFRCQPGFVMKGPRRVKCQALNKWEPELPSCSRVCQPPPEILHGEHTPSHQDNFSPGQEVFYSCEPGYDLRGAASLHCTPQGDWSPEAPRCAVKSCDDFLGQLPHGRVLFPLNLQLGAKVSFVCDEGFRLKGSSVSHCVLVGMRSLWNNSVPVCEHIFCPNPPAILNGRHTGTPSGDIPYGKEISYTCDPHPDRGMTFNLIGESTIRCTSDPHGNGVWSSPAPRCELSVR

SEQ ID NO: 48 - protein, 1537 aa, Artificial Sequence
  amino acid sequence of truncated mature soluble complement receptor 1 conjugated to HSA (sCR1(939)-GS13-HSA) with N-terminal endogenous signal peptide
MGASSPRSPEPVGPPAPGLPFCCGGSLLAVVVLLALPVAWGQCNAPEWLPFARPTNLTDEFEFPIGTYLNYECRPGYSGRPFSIICLKNSVWTGAKDRCRRKSCRNPPDPVNGMVHVIKGIQFGSQIKYSCTKGYRLIGSSSATCIISGDTVIWDNETPICDRIPCGLPPTITNGDFISTNRENFHYGSVVTYRCNPGSGGRKVFELVGEPSIYCTSNDDQVGIWSGPAPQCIIPNKCTPPNVENGILVSDNRSLFSLNEVVEFRCQPGFVMKGPRRVKCQALNKWEPELPSCSRVCQPPPDVLHAERTQRDKDNFSPGQEVFYSCEPGYDLRGAASMRCTPQGDWSPAAPTCEVKSCDDFMGQLLNGRVLFPVNLQLGAKVDFVCDEGFQLKGSSASYCVLAGMESLWNSSVPVCEQIFCPSPPVIPNGRHTGKPLEVFPFGKTVNYTCDPHPDRGTSFDLIGESTIRCTSDPQGNGVWSSPAPRCGILGHCQAPDHFLFAKLKTQTNASDFPIGTSLKYECRPEYYGRPFSITCLDNLVWSSPKDVCKRKSCKTPPDPVNGMVHVITDIQVGSRINYSCTTGHRLIGHSSAECILSGNAAHWSTKPPICQRIPCGLPPTIANGDFISTNRENFHYGSVVTYRCNPGSGGRKVFELVGEPSIYCTSNDDQVGIWSGPAPQCIIPNKCTPPNVENGILVSDNRSLFSLNEVVEFRCQPGFVMKGPRRVKCQALNKWEPELPSCSRVCQPPPDVLHAERTQRDKDNFSPGQEVFYSCEPGYDLRGAASMRCTPQGDWSPAAPTCEVKSCDDFMGQLLNGRVLFPVNLQLGAKVDFVCDEGFQLKGSSASYCVLAGMESLWNSSVPVCEQIFCPSPPVIPNGRHTGKPLEVFPFGKAVNYTCDPHPDRGTSFDLIGESTIRCTSDPQGNGVWSSPAPRCGIGSGGSGGSGGSGSDAHKSEVAHRFKDLGEENFKALVLIAFAQYLQQCPFEDHVKLVNEVTEFAKTCVADESAENCDKSLHTLFGDKLCTVATLRETYGEMADCCAKQEPERNECFLQHKDDNPNLPRLVRPEVDVMCTAFHDNEETFLKKYLYEIARRHPYFYAPELLFFAKRYKAAFTECCQAADKAACLLPKLDELRDEGKASSAKQRLKCASLQKFGERAFKAWAVARLSQRFPKAEFAEVSKLVTDLTKVHTECCHGDLLECADDRADLAKYICENQDSISSKLKECCEKPLLEKSHCIAEVENDEMPADLPSLAADFVESKDVCKNYAEAKDVFLGMFLYEYARRHPDYSVVLLLRLAKTYETTLEKCCAAADPHECYAKVFDEFKPLVEEPQNLIKQNCELFEQLGEYKFQNALLVRYTKKVPQVSTPTLVEVSRNLGKVGSKCCKHPEAKRMPCAEDYLSVVLNQLCVLHEKTPVSDRVTKCCTESLVNRRPCFSALEVDETYVPKEFNAETFTFHADICTLSEKERQIKKQTALVELVKHKPKATKEQLKAVMDDFAAFVEKCCKADDKETCFAEEGKKLVAASQAALGL

SEQ ID NO: 49 - protein, 1140 aa, Artificial Sequence
  amino acid sequence of truncated mature soluble complement receptor 1 conjugated to IgG4 Fc (sCR1(939)-IgG4 Fc)) with N-terminal endogenous signal peptide
MGASSPRSPEPVGPPAPGLPFCCGGSLLAVVVLLALPVAWGQCNAPEWLPFARPTNLTDEFEFPIGTYLNYECRPGYSGRPFSIICLKNSVWTGAKDRCRRKSCRNPPDPVNGMVHVIKGIQFGSQIKYSCTKGYRLIGSSSATCIISGDTVIWDNETPICDRIPCGLPPTITNGDFISTNRENFHYGSVVTYRCNPGSGGRKVFELVGEPSIYCTSNDDQVGIWSGPAPQCIIPNKCTPPNVENGILVSDNRSLFSLNEVVEFRCQPGFVMKGPRRVKCQALNKWEPELPSCSRVCQPPPDVLHAERTQRDKDNFSPGQEVFYSCEPGYDLRGAASMRCTPQGDWSPAAPTCEVKSCDDFMGQLLNGRVLFPVNLQLGAKVDFVCDEGFQLKGSSASYCVLAGMESLWNSSVPVCEQIFCPSPPVIPNGRHTGKPLEVFPFGKTVNYTCDPHPDRGTSFDLIGESTIRCTSDPQGNGVWSSPAPRCGILGHCQAPDHFLFAKLKTQTNASDFPIGTSLKYECRPEYYGRPFSITCLDNLVWSSPKDVCKRKSCKTPPDPVNGMVHVITDIQVGSRINYSCTTGHRLIGHSSAECILSGNAAHWSTKPPICQRIPCGLPPTIANGDFISTNRENFHYGSVVTYRCNPGSGGRKVFELVGEPSIYCTSNDDQVGIWSGPAPQCIIPNKCTPPNVENGILVSDNRSLFSLNEVVEFRCQPGFVMKGPRRVKCQALNKWEPELPSCSRVCQPPPDVLHAERTQRDKDNFSPGQEVFYSCEPGYDLRGAASMRCTPQGDWSPAAPTCEVKSCDDFMGQLLNGRVLFPVNLQLGAKVDFVCDEGFQLKGSSASYCVLAGMESLWNSSVPVCEQIFCPSPPVIPNGRHTGKPLEVFPFGKAVNYTCDPHPDRGTSFDLIGESTIRCTSDPQGNGVWSSPAPRCGIESKYGPPCPPCPAPEFLGGPSVFLFPPKPKDTLMISRTPEVTCVVVDVSQEDPEVQFNWYVDGVEVHNAKTKPREEQFNSTYRVVSVLTVLHQDWLNGKEYKCKVSNKGLPSSIEKTISKAKGQPREPQVYTLPPSQEEMTKNQVSLTCLVKGFYPSDAIVEWESNGQPENNYKTTPPVLDSDGSFFLYSRLTVDKSRWQE

SEQ ID NO: 50 - protein, 1146 aa, Artificial Sequence
  amino acid sequence of truncated mature soluble complement receptor 1 conjugated to IgG4 Fc (IgG4 Fc-sCR1(939)) with N-terminal exogenous signal peptide
MGWSCIILFLVATATGVHSESKYGPPCPSCPAPEFLGGPSVFLFPPKPKDTLMISRTPEVTCVVVDVSQEDPEVQFNWYVDGVEVHNAKTKPREEQFNSTYRVVSVLTVLHQDWLNGKEYKCKVSNKGLPSSIEKTISKAKGQPREPQVYTLPPSQEEMTKNQVSLTCLVKGFYPSDIAVEWESNGQPENNYKTTPPVLDSDGSFFLYSRLTVDKSRWQEGNVFSCSVMHEALHNHYTQKSLSLSLGKQCNAPEWLPFARPTNLTDEFEFPIGTYLNYECRPGYSGRPFSIICLKNSVWTGAKDRCRRKSCRNPPDPVNGMVHVIKGIQFGSQIKYSCTKGYRLIGSSSATCIISGDTVIWDNETPICDRIPCGLPPTITNGDFISTNRENFHYGSVVTYRCNPGSGGRKVFELVGEPSIYCTSNDDQVGIWSGPAPQCIIPNKCTPPNVENGILVSDNRSLFSLNEVVEFRCQPGFVMKGPRRVKCQALNKWEPELPSCSRVCQPPPDVLHAERTQRDKDNFSPGQEVFYSCEPGYDLRGAASMRCTPQGDWSPAAPTCEVKSCDDFMGQLLNGRVLFPVNLQLGAKVDFVCDEGFQLKGSSASYCVLAGMESLWNSSVPVCEQIFCPSPPVIPNGRHTGKPLEVFPFGKTVNYTCDPHPDRGTSFDLIGESTIRCTSDPQGNGVWSSPAPRCGILGHCQAPDHFLFAKLKTQTNASDFPIGTSLKYECRPEYYGRPFSITCLDNLVWSSPKDVCKRKSCKTPPDPVNGMVHVITDIQVGSRINYSCTTGHRLIGHSSAECILSGNAAHWSTKPPICQRIPCGLPPTIANGDFISTNRENFHYGSVVTYRCNPGSGGRKVFELVGEPSIYCTSNDDQVGIWSGPAPQCIIPNKCTPPNVENGILVSDNRSLFSLNEVVEFRCQPGFVMKGPRRVKCQALNKWEPELPSCSRVCQPPPDVLHAERTQRDKDNFSPGQEVFYSCEPGYDLRGAASMRCTPQGDWSPAAPTCEVKSCDDFMGQLLNGRVLFPVNLQLGAKVDFVCDEGFQLKGSSASYCVLAGMESLWNSSVPVCEQIFCPSPPVIPNGRHTGKPLEVFPFGKAVNYTCDPHPDRGTSFDLIGESTIRCTSDPQGNGVWSSPAPRCGI

SEQ ID NO: 51 - protein, 1977 aa, Artificial Sequence
  amino acid sequence of truncated mature soluble complement receptor 1 conjugated to HSA (sCR1(1392)-HSA
MGASSPRSPEPVGPPAPGLPFCCGGSLLAVVVLLALPVAWGQCNAPEWLPFARPTNLTDEFEFPIGTYLNYECRPGYSGRPFSIICLKNSVWTGAKDRCRRKSCRNPPDPVNGMVHVIKGIQFGSQIKYSCTKGYRLIGSSSATCIISGDTVIWDNETPICDRIPCGLPPTITNGDFISTNRENFHYGSVVTYRCNPGSGGRKVFELVGEPSIYCTSNDDQVGIWSGPAPQCIIPNKCTPPNVENGILVSDNRSLFSLNEVVEFRCQPGFVMKGPRRVKCQALNKWEPELPSCSRVCQPPPDVLHAERTQRDKDNFSPGQEVFYSCEPGYDLRGAASMRCTPQGDWSPAAPTCEVKSCDDFMGQLLNGRVLFPVNLQLGAKVDFVCDEGFQLKGSSASYCVLAGMESLWNSSVPVCEQIFCPSPPVIPNGRHTGKPLEVFPFGKTVNYTCDPHPDRGTSFDLIGESTIRCTSDPQGNGVWSSPAPRCGILGHCQAPDHFLFAKLKTQTNASDFPIGTSLKYECRPEYYGRPFSITCLDNLVWSSPKDVCKRKSCKTPPDPVNGMVHVITDIQVGSRINYSCTTGHRLIGHSSAECILSGNAAHWSTKPPICQRIPCGLPPTIANGDFISTNRENFHYGSVVTYRCNPGSGGRKVFELVGEPSIYCTSNDDQVGIWSGPAPQCIIPNKCTPPNVENGILVSDNRSLFSLNEVVEFRCQPGFVMKGPRRVKCQALNKWEPELPSCSRVCQPPPDVLHAERTQRDKDNFSPGQEVFYSCEPGYDLRGAASMRCTPQGDWSPAAPTCEVKSCDDFMGQLLNGRVLFPVNLQLGAKVDFVCDEGFQLKGSSASYCVLAGMESLWNSSVPVCEQIFCPSPPVIPNGRHTGKPLEVFPFGKAVNYTCDPHPDRGTSFDLIGESTIRCTSDPQGNGVWSSPAPRCGILGHCQAPDHFLFAKLKTQTNASDFPIGTSLKYECRPEYYGRPFSITCLDNLVWSSPKDVCKRKSCKTPPDPVNGMVHVITDIQVGSRINYSCTTGHRLIGHSSAECILSGNTAHWSTKPPICQRIPCGLPPTIANGDFISTNRENFHYGSVVTYRCNLGSRGRKVFELVGEPSIYCTSNDDQVGIWSGPAPQCIIPNKCTPPNVENGILVSDNRSLFSLNEVVEFRCQPGFVMKGPRRVKCQALNKWEPELPSCSRVCQPPPEILHGEHTPSHQDNFSPGQEVFYSCEPGYDLRGAASLHCTPQGDWSPEAPRCAVKSCDDFLGQLPHGRVLFPLNLQLGAKVSFVCDEGFRLKGSSVSHCVLVGMRSLWNNSVPVCEHIFCPNPPAILNGRHTGTPSGDIPYGKEISYTCDPHPDRGMTFNLIGESTIRCTSDPHGNGVWSSPAPRCELSVRDAHKSEVAHRFKDLGEENFKALVLIAFAQYLQQCPFEDHVKLVNEVTEFAKTCVADESAENCDKSLHTLFGDKLCTVATLRETYGEMADCCAKQEPERNECFLQHKDDNPNLPRLVRPEVDVMCTAFHDNEETFLKKYLYEIARRHPYFYAPELLFFAKRYKAAFTECCQAADKAACLLPKLDELRDEGKASSAKQRLKCASLQKFGERAFKAWAVARLSQRFPKAEFAEVSKLVTDLTKVHTECCHGDLLECADDRADLAKYICENQDSISSKLKECCEKPLLEKSHCIAEVENDEMPADLPSLAADFVESKDVCKNYAEAKDVFLGMFLYEYARRHPDYSVVLLLRLAKTYETTLEKCCAAADPHECYAKVFDEFKPLVEEPQNLIKQNCELFEQLGEYKFQNALLVRYTKKVPQVSTPTLVEVSRNLGKVGSKCCKHPEAKRMPCAEDYLSVVLNQLCVLHEKTPVSDRVTKCCTESLVNRRPCFSALEVDETYVPKEFNAETFTFHADICTLSEKERQIKKQTALVELVKHKPKATKEQLKAVMDDFAAFVEKCCKADDKETCFAEEGKKLVAASQAALGL